European Patent Specification EP 3 690 052 B1, published April 19, 2023. Title: Chimeric promoter for use in metabolic engineering. Applicant: Clariant Produkte (Deutschland) GmbH. The sequence listing filed with the application follows.

SEQUENCE LISTING (138 sequences)

SEQ ID NO: 1 - DNA, 701 bp, Artificial Sequence
  chimeric promoter
aaatgatcacaaatgtgattgatgatttgacacgactagaaaagagaacgaaaaagggaaattccatgtcacgtgcgttggcacgtgacatggaatatcgaagaaagaaaaaaaaaaacgatctcgtcctagtggaagcccagagtctggtccccccggagtcttcccaaaacaagaagctgacacatgttgacacagaacaccccacagcaaatgcaccacgctacgtagatcaggaagcttaactctagcgacctgtcgctcgccccacagaacctcacccgagaaccacacattacacgccgccagctcccactatactcatcttgcttcccttaagcgttctcacgattcgttcgctggataattatcttcttccgtctatcttcttctaaattgatcagtatcataatatggaaaaaaaggttgttcgtgaatttttcctccattcaattcatatataataagaacaatgaattgcatacttcccaaatcttgataattcgttttaatatctatcagtagttgtttatattcaattatatcttgtgtatacaaaaccatcatccaaaaaccaatccaagtttcgtttgacttataaccaatagtaccaaaaattaaaccttaattttgaagtactttataatttaaacttaatacgaattaaaccaaaaaacccacaacacgtaaaagaaattaca

SEQ ID NO: 2 - DNA, 700 bp, Artificial Sequence
  chimeric promoter
ttactttcccggataatttcgaagaggatattacccgcttacgccagatgcatgcgaacttgatgcagcacatgaagagacaatcaacagagaccccaggaaatcttgaagaacaacagaaacacatcaatgatatcgtagataccattgagagatataactgaataaatacttcaaatcacgtgatgaatcacgtgccacaattaccctgactttttgtttacgcagcaaacatgcagcatccactaacttcagagattcctgtaagataagtggttcgttattttccggattccaattttggtggtgctccgaaaagtggaagctcgtgatcctacatgctcacgaaacccatcatcatgcaatccacattaaaggaagggaaaaggatattgaacttttgactatttagtataaatgaaaactactttgtaagcttggacagaggaataatttctgattcgtgcttctgcttctactgacttgcaaatttacatataaatatacgtcaaaaggggattcattaattagaaaattctctttttcaatagttgctattcattatcaatctattcaactcaattggttattattttcatctttttgtcatcctaaaccatcaacaatatttaaatatatctgttgctacattaagagttacttcagaaataacaaaaaaatcgatcaagaattaataaaa

SEQ ID NO: 3 - DNA, 710 bp, Artificial Sequence
  chimeric promoter
taatatttatctggataattgtgagtgcttgaattaccttctatctcacgtgatttgattctattggacaaaaagggaaagaccctcctgagagattaaaataattacccggatctaagagatttcacgttaaaatatacatctccttccgagtactcttagcttccactattttaacggggctattcatgcgttccgggtaatgaggtgttcccggagccaaaaatcatcttcctttatcagaaagacacgttcacaatccaggcaccccacagagaaaaaaaaaagaagaagcccggaagctggcacgccatcatcaaccaccgctcggtttacacgcatcccaactgtcttttttttctggaatcctggataattatcttcttccgtctatcttcttctaaattgatcagtatcataatatggaaaaaaaggttgttcgtgaatttttcctccattcaattcatatataataagaacaatgaattgctctttatatatatatattctctggtgaaggttcttgatcaattgcttcttccaattggtatttcgattgtattcttgagtcacgtagaaaggaatttgtgattagggtttaatcgctgaattctgaagtgaccttttaactgaccgtaaagtacaataaaaggttttaaagttctgttaagatagattctaaaacagaaataaaaagacaaatatcagaa

SEQ ID NO: 4 - DNA, 130 bp, Kluyveromyces lactis
  promoter fragment
cagaaagacacgttcacaatccaggcaccccacagagaaaaaaaaaagaagaagcccggaagctggcacgccatcatcaaccaccgctcggtttacacgcatcccaactgtcttttttttctggaatcct

SEQ ID NO: 5 - DNA, 120 bp, Kluyveromyces lactis
  promoter fragment
ggataattatcttcttccgtctatcttcttctaaattgatcagtatcataatatggaaaaaaaggttgttcgtgaatttttcctccattcaattcatatataataagaacaatgaattgc

SEQ ID NO: 6 - DNA, 340 bp, Kluyveromyces lactis
  promoter fragment
ggataattatcttcttccgtctatcttcttctaaattgatcagtatcataatatggaaaaaaaggttgttcgtgaatttttcctccattcaattcatatataataagaacaatgaattgcatacttcccaaatcttgataattcgttttaatatctatcagtagttgtttatattcaattatatcttgtgtatacaaaaccatcatccaaaaaccaatccaagtttcgtttgacttataaccaatagtaccaaaaattaaaccttaattttgaagtactttataatttaaacttaatacgaattaaaccaaaaaacccacaacacgtaaaagaaattaca

SEQ ID NO: 7 - DNA, 270 bp, Kluyveromyces lactis
  promoter fragment
ttacgcagcaaacatgcagcatccactaacttcagagattcctgtaagataagtggttcgttattttccggattccaattttggtggtgctccgaaaagtggaagctcgtgatcctacatgctcacgaaacccatcatcatgcaatccacattaaaggaagggaaaaggatattgaacttttgactatttagtataaatgaaaactactttgtaagcttggacagaggaataatttctgattcgtgcttctgcttctactgacttgcaaa

SEQ ID NO: 8 - DNA, 220 bp, Kluyveromyces lactis
  promoter fragment
ttactttcccggataatttcgaagaggatattacccgcttacgccagatgcatgcgaacttgatgcagcacatgaagagacaatcaacagagaccccaggaaatcttgaagaacaacagaaacacatcaatgatatcgtagataccattgagagatataactgaataaatacttcaaatcacgtgatgaatcacgtgccacaattaccctgactttttgt

SEQ ID NO: 9 - DNA, 220 bp, Kluyveromyces lactis
  promoter fragment
tctttatatatatatattctctggtgaaggttcttgatcaattgcttcttccaattggtatttcgattgtattcttgagtcacgtagaaaggaatttgtgattagggtttaatcgctgaattctgaagtgaccttttaactgaccgtaaagtacaataaaaggttttaaagttctgttaagatagattctaaaacagaaataaaaagacaaatatcagaa

SEQ ID NO: 10 - DNA, 361 bp, Kluyveromyces lactis
  promoter fragment
aaatgatcacaaatgtgattgatgatttgacacgactagaaaagagaacgaaaaagggaaattccatgtcacgtgcgttggcacgtgacatggaatatcgaagaaagaaaaaaaaaaacgatctcgtcctagtggaagcccagagtctggtccccccggagtcttcccaaaacaagaagctgacacatgttgacacagaacaccccacagcaaatgcaccacgctacgtagatcaggaagcttaactctagcgacctgtcgctcgccccacagaacctcacccgagaaccacacattacacgccgccagctcccactatactcatcttgcttcccttaagcgttctcacgattcgttcgct

SEQ ID NO: 11 - DNA, 210 bp, Kluyveromyces lactis
  promoter fragment
tttacatataaatatacgtcaaaaggggattcattaattagaaaattctctttttcaatagttgctattcattatcaatctattcaactcaattggttattattttcatctttttgtcatcctaaaccatcaacaatatttaaatatatctgttgctacattaagagttacttcagaaataacaaaaaaatcgatcaagaattaataaaa

SEQ ID NO: 12 - DNA, 240 bp, Kluyveromyces lactis
  promoter fragment
taatatttatctggataattgtgagtgcttgaattaccttctatctcacgtgatttgattctattggacaaaaagggaaagaccctcctgagagattaaaataattacccggatctaagagatttcacgttaaaatatacatctccttccgagtactcttagcttccactattttaacggggctattcatgcgttccgggtaatgaggtgttcccggagccaaaaatcatcttcctttat

SEQ ID NO: 13 - DNA, 1329 bp, Artificial Sequence
  xylose isomerase gene
atgaaggaattcttcccaggtatttctccagttaagttcgaaggtagagactctaagaacccattgtctttcaagtactacgacgctaagagagttattatgggtaagaccatggaagaacacttgtctttcgctatggcttggtggcacaacttgtgtgcttgtggtgttgacatgttcggtcaaggtaccgttgacaagtctttcggtgaatcttctggtaccatggaacacgctagagctaaggttgacgctggtattgaattcatgaagaagttgggtattaagtactactgtttccacgacaccgacattgttccagaagaccaagaagacattaacgttaccaacgctagattggacgaaattaccgactacattttggaaaagaccaaggacaccgacattaagtgtttgtggaccacctgtaacatgttctctaacccaagattcatgaacggtgctggttcttctaactctgctgacgttttctgtttcgctgctgctcaagctaagaagggtttggaaaacgctgttaagttgggtgctaagggtttcgttttctggggtggtagagaaggttacgaaaccttgttgaacaccgacatgaagttggaagaagaaaacattgctaccttgttcaccatgtgtagagactacggtagatctattggtttcatgggtgacttctacattgaaccaaagccaaaggaaccaatgaagcaccaatacgacttcgacgctgctaccgctattggtttcttgagaaagtacggtttggacaaggacttcaagttgaacattgaagctaaccacgctaccttggctggtcacaccttccaacacgaattgagagtttgtgctgttaacggtatgatgggttctgttgacgctaaccaaggtgacaccttgttgggttgggacaccgaccaattcccaaccaacgtttacgacaccaccttggctatgtacgaaattttgaaggctggtggtttgagaggtggtttgaacttcgactctaagaacagaagaccatctaacaccgctgacgacatgttctacggtttcattgctggtatggacaccttcgctttgggtttgattaaggctgctgaaattattgaagacggtagaattgacgacttcgttaaggaaagatacgcttcttacaactctggtattggtaagaagattagaaacagaaaggttaccttgattgaatgtgctgaatacgctgctaagttgaagaagccagaattgccagaatctggtagacaagaatacttggaatctgttgtcaacaacattttgttcggtggttctggttaa

SEQ ID NO: 14 - DNA, 600 bp, Saccharomyces cerevisiae
  promoter
gggccagaaaaaggaagtgtttccctccttcttgaattgatgttaccctcataaagcacgtggcctcttatcgagaaagaaattaccgtcgctcgtgatttgtttgcaaaaagaacaaaactgaaaaaacccagacacgctcgacttcctgtcttcctattgattgcagcttccaatttcgtcacacaacaaggtcctagcgacggctcacaggttttgtaacaagcaatcgaaggttctggaatggcgggaaagggtttagtaccacatgctatgatgcccactgtgatctccagagcaaagttcgttcgatcgtactgttactctctctctttcaaacagaattgtccgaatcgtgtgacaacaacagcctgttctcacacactcttttcttctaaccaagggggtggtttagtttagtagaacctcgtgaaacttacatttacatatatataaacttgcataaattggtcaatgcaagaaatacatatttggtcttttctaattcgtagtttttcaagttcttagatgctttctttttctcttttttacagatcatcaaggaagtaattatctactttttacaacaaatataaaaca

SEQ ID NO: 15 - protein, 442 aa, Artificial Sequence
  xylose isomerase
MKEFFPGISPVKFEGRDSKNPLSFKYYDAKRVIMGKTMEEHLSFAMAWWHNLCACGVDMFGQGTVDKSFGESSGTMEHARAKVDAGIEFMKKLGIKYYCFHDTDIVPEDQEDINVTNARLDEITDYILEKTKDTDIKCLWTTCNMFSNPRFMNGAGSSNSADVFCFAAAQAKKGLENAVKLGAKGFVFWGGREGYETLLNTDMKLEEENIATLFTMCRDYGRSIGFMGDFYIEPKPKEPMKHQYDFDAATAIGFLRKYGLDKDFKLNIEANHATLAGHTFQHELRVCAVNGMMGSVDANQGDTLLGWDTDQFPTNVYDTTLAMYEILKAGGLRGGLNFDSKNRRPSNTADDMFYGFIAGMDTFALGLIKAAEIIEDGRIDDFVKERYASYNSGIGKKIRNRKVTLIECAEYAAKLKKPELPESGRQEYLESVVNNILFGGSG

SEQ ID NO: 16 - DNA, 800 bp, Kluyveromyces lactis
  promoter
acagttgatcctattactttttttttattttttgtccctccgggatggcaagagggacaaagaagaatcttcgttcttctttcttgttctcaacttcccagcttccgtgtgattaccctccgggacaacagaaaaactggcattcggtatcccgggaatctgctgagaaggaaagaaaacgaaaaaaaaattgtacatttgtgtcacattatgaattacaggaagtcagaaaacaggcagcacatgtctcgcacatgcatgtccatcagacgagacattatgagacatgcacgcgtgtgagagacatagcaaaagtctctccagtacacacagaaagacacgttcacaatccaggcaccccacagagaaaaaaaaaagaagaagcccggaagctggcacgccatcatcaaccaccgctcggtttacacgcatcccaactgtcttttttttctggaatcctataataactggcatctggaaatcacgttgtatgttgcaccatagtgactggctgtctgactagcaaacattgattccctgattcccatttggctcaattttgatgagaaacagttgattgattcttgtcaatttttttttctttggaccaccaccaaccaattgacattgaagtactttcccatgatttgaggttatataaaaggacgttcaaatcactttcaaggttaattcagttttgtcaattgatttaagttcaattgttaacaaatttaatttaattcgaaacaaaccaaaccaattcatttgaattaacaaaccaacccacaaaacaaaaaaac

SEQ ID NO: 17 - DNA, 800 bp, Kluyveromyces lactis
  promoter
cgtgagaggtggcctgacagagaactgaacaaaaaaaaaaaaaagaaaaagaaagccaaacaaaatccgcagctggaaccttaattactggacgcccgacttcttgaaaaacacactggcattaaacaagaagctaccagaatgtgttcacgtacaggcagttggtgttctgtgttcttacaaaaaagtttcgccttagtcgcagtgagaacgtgcaataagctgatctactcaacgcaactgacaaagactagcaataactgccacatgatattctcaaaacccactttgcgatgcaattgagcgatgtataatcacaccaaccaacatacgtgtttctagaaattggcagttttgcccggcctgattgcctagatagtgcagtggcagttggaacacctgtcgcaagctctcttcatatcatcatctttatccctcttttctgagtgatgttctgtctggataattatcttcttccgtctatcttcttctaaattgatcagtatcataatatggaaaaaaaggttgttcgtgaatttttcctccattcaattcatatataataagaacaatgaattgcatacttcccaaatcttgataattcgttttaatatctatcagtagttgtttatattcaattatatcttgtgtatacaaaaccatcatccaaaaaccaatccaagtttcgtttgacttataaccaatagtaccaaaaattaaaccttaattttgaagtactttataatttaaacttaatacgaattaaaccaaaaaacccacaacacgtaaaagaaattaca

SEQ ID NO: 18 - DNA, 800 bp, Kluyveromyces lactis
  promoter
ccagatatccaatggtctccaaagttcaatcaaggtaaaatgaagaatctcgccttcatcaaggaccctgatggatactccatcgaagtcgtcccatacggattgggcgtttgaagagcaccaaactctcatctatttatttgaaatgtaaatgcaaatttatgtatcgttgtatacaatattcgatatgacaccgttcaatcgccatattacagccataactgccggtaatactgataaagatatccttttgaagtgacatgaaagcacgtgactgagattaatataactcttcacatttttttttttttaatttttcattacgcagcaaacatgcagcatccactaacttcagagattcctgtaagataagtggttcgttattttccggattccaattttggtggtgctccgaaaagtggaagctcgtgatcctacatgctcacgaaacccatcatcatgcaatccacattaaaggaagggaaaaggatattgaacttttgactatttagtataaatgaaaactactttgtaagcttggacagaggaataatttctgattcgtgcttctgcttctactgacttgcaaaccagtaaacaagttactgcattaatcagtaataatctgcgtatagcgaaacttgtaaccagtttcctcgtaacaaggttagcagaagaatttgcaagaggatcaagttgataaagacgtatatttaggtctctgcacgttttcaaacttttaagcgagaatcaaacgattacaaaaaggaaaatattgatacaagtaataataaactgca

SEQ ID NO: 19 - DNA, 800 bp, Kluyveromyces lactis
  promoter
gtacatgctacaccaaaagtggatgacaaggataggatatggacagatatagatacactagatgatgtgaaaagaatggccagagagggcaatactggccttactttcccggataatttcgaagaggatattacccgcttacgccagatgcatgcgaacttgatgcagcacatgaagagacaatcaacagagaccccaggaaatcttgaagaacaacagaaacacatcaatgatatcgtagataccattgagagatataactgaataaatacttcaaatcacgtgatgaatcacgtgccacaattaccctgactttttgttgagtattagtggaagctaaggtttccaaggaccaccggtttcttctacgtgcctttcactatttgtttactggatggtgcgaaacaaataaaaaaagcggaagctgacagaaattacaagttgttccgaataacgatgggatatacgaattgatgattgaacgtagtatggaaaataataggaacgttgagaaaaaaaaggatttggtattttccatcacctgcgaatttgagggaaatggttaacttaaatcgtggattctttatatatatatattctctggtgaaggttcttgatcaattgcttcttccaattggtatttcgattgtattcttgagtcacgtagaaaggaatttgtgattagggtttaatcgctgaattctgaagtgaccttttaactgaccgtaaagtacaataaaaggttttaaagttctgttaagatagattctaaaacagaaataaaaagacaaatatcagaa

SEQ ID NO: 20 - DNA, 801 bp, Kluyveromyces lactis
  promoter
ggtaatccaattgtctgtctgctcagtttagcacatgtatagtacgttgcacatagtctacaatattcagcattcagcattcagtatacagcatatggctaaatgatcacaaatgtgattgatgatttgacacgactagaaaagagaacgaaaaagggaaattccatgtcacgtgcgttggcacgtgacatggaatatcgaagaaagaaaaaaaaaaacgatctcgtcctagtggaagcccagagtctggtccccccggagtcttcccaaaacaagaagctgacacatgttgacacagaacaccccacagcaaatgcaccacgctacgtagatcaggaagcttaactctagcgacctgtcgctcgccccacagaacctcacccgagaaccacacattacacgccgccagctcccactatactcatcttgcttcccttaagcgttctcacgattcgttcgctgcccttcttcaagagtcttctgattctaattctcattcgaaatcctctacagttaatgaattgcttgacatgacattcattgtctcatggttttggctttttggcttttgtcttttaaagctatatcaactttacatataaatatacgtcaaaaggggattcattaattagaaaattctctttttcaatagttgctattcattatcaatctattcaactcaattggttattattttcatctttttgtcatcctaaaccatcaacaatatttaaatatatctgttgctacattaagagttacttcagaaataacaaaaaaatcgatcaagaattaataaaa

SEQ ID NO: 21 - DNA, 710 bp, Kluyveromyces lactis
  promoter
taatatttatctggataattgtgagtgcttgaattaccttctatctcacgtgatttgattctattggacaaaaagggaaagaccctcctgagagattaaaataattacccggatctaagagatttcacgttaaaatatacatctccttccgagtactcttagcttccactattttaacggggctattcatgcgttccgggtaatgaggtgttcccggagccaaaaatcatcttcctttatttcgcatcctataatgacgaaatgcaaaaacaccatgcgggcacgaagttgggcttcttctttttccggctcacagaataggacgctgccgattgtcaaagtcaatcagtgtgctgtctgacaacctgatagttggttccatggttttcagtaacatacgcatacctcctgctcactttgactataggaaacagaccatggtgatttccattcgataatgtttctaaacacttgaactttcatgtattctttcgaaccttcttcgtatttttgttttatgtatatatatatatatatatgtgtataaatttcatagaaaggtttaaagatcaattgatactcgtaaccacttctttatcagtcgaattattggtttattggttttgtttcaaggaaaaccaaggaacagcatcatcaattgattatcattcccctatttcaactaacacacacataactcacatacaatc

SEQ ID NO: 22 - protein, 342 aa, Saccharomyces cerevisiae
MKDNQENHDQKPFIILGDKNKFEATIAKVGATLVDLKVNGQSVVLGYPDVKGYLNDPGNLVGANVGRYANRIYKGVFNTPDGAHQLTVNNCGNANHSSISCFNRKTFVASPVENSSRDVYIAKLTLLDDHTVPNEFPGDLEVTVTYTLNVAEMTLDLDYRAHLVKGDATPINMTNHTYFNLNKTRNEESIIGTEINICSDKSLEVTEGALIPTGKIIKRDIATFQSAHPTTLGSKAPVYDFCFIVDANKDLRSTDSTSVNKLVPVFKAYHPESNIRLQVSTTEPTVHFYTGDSLGGKFVPRSGFAVEQGRYIDAINRSEWRNCVLLKRGEVYTSKTQYCFKN

SEQ ID NO: 23 - protein, 359 aa, Saccharomyces cerevisiae
MGSKNTLLVFHLKGVKTDLAGAVNDYENRFITIGAGSKFEATIANLGATLVDLKVNGQSVVLGYSRAEDYNSDGGNYIGATVGRFANRIKEGLFTLQDGTHKLTVDNCDNTNHSSISSFHVKKFLGPLIENPSDEIYTAEFLLLDDHSIPNEFPGDLEVIVKFTLNIAEMSLKFSYQAQLINGEATPINMTSHTYFNLNKFHNEQSISGTEVRVCSTKSLEVSEGALIPTGKVIDRDVATFDSAGPTTLGGDGPTYDYCFISDENKGLKSPDSRSQNELRPVLKAYHPESKITLEVSTTEPSFVLYSGDNLFGKFIPRQGFCVEQGRYIDAINRDDWKDCVLLKRGDVYTSETQYRFEN

SEQ ID NO: 24 - protein, 341 aa, Saccharomyces cerevisiae
MSNNKAGGEYEVITIGDAKKLQATISELGATLLDLKVNNESIVLGYPDIHGYISDGYNYIGATVGRYANRIYKGMFSMEDGPHQLTVNNCGNTNHSSISSFHLKKYKASKVQNPLDDLYIVEFTLLDDRTLPNEFPGDLAVNLKYTLNVADMTLDLEYEAKLVSGEATPINMTNHTYFNLNKTMDKKSISGTEVRLCSDKSLEVSEGALIPTGKIVQRKIATFDSSKPTILQDDGPIYDYAFIVDENKNLKTTDSVSVNKLVPAFKAYHPASRLSLEVSTTEPTVLFYTGDNLCDGFTPRSGFAVEQGRYVDAINRDGWRDCVLLRRGEVYTSKTRYRFAV

SEQ ID NO: 25 - protein, 360 aa, Saccharomyces cerevisiae x Saccharomyces kudriavzevii
MSNDGQQKKLATIDNKLEMTNSNTENKYKVITIGDEKRFQATIAPLGATLVDLKVNNQSVVQGYSNVQDYLTDGNMMGATVGRYANRIAKGVFSLEDGPHKLTVNNCGNTNHSSISSLNLKQYRASPVENPSKDVFVVEFKLLDDHTQPNPNEFPGDLEVTVKYTLNVAEMTLGMKYQAQLVRGDATPINMTNHSYFNLNKTKNEKSISGTEVKVCSNKSLEVTEGALLPTEKIIERKIATFDSAKPTVLHDDAPVFDCTFIIDANKDLHTTDSVSVNKLVPVFKAYHPESRITFEVSTTEPTVHLYTGDNLCGKFTPRSGFAVQQGRYVDAINHDKWRDCVLLKRGEVYTSETQYRFGI

SEQ ID NO: 26 - protein, 342 aa, Saccharomyces cerevisiae
MSNSNGDNKYGVITIGDEKKFQATIAPLGATLVDLKVNGQSVVQGYSNVQDYLTDGNMMGATVGRYANRIAKGVFSLDDGPHKLTVNNCGNTNHSSISSLNLKQYKASPVENPSKGVYVVEFKLLDDHTQPNPNEFPGDLEVTVKYTLNVAEMTLDMEYQAQLVRGDATPINMTNHSYFNLNKVKSEKSIRGTEVKVCSNKSLEVTEGALLPTGKIIERNIATFDSTKPTVLHEDTPVFDCTFIIDANKDLKTTDSVSVNKLVPVFKAYHPESHIKFEVSTTEPTVHLYTGDNLCGKFVPRSGFAVQQGRYVDAINRDEWRGCVLLKRGEVYTSKTQYKFDI

SEQ ID NO: 27 - protein, 334 aa, Lactococcus lactis
MTFTISKESLPFRADKSISQITLSNERLTIVVHDYGARAHQLLTPDKNGTFENILLSKNDSETYANDGGYYGVICGPVAGRISGATYDSVSLEANEGKNNLHSGSHGWERQFWSYETFETASSLGIKLSLRDEESGFPGQIQAEVTYKLTDNKLEVTISGLSVTDTVFNPAWHPYFNLSAELSTTHEHFIQANVDFLVETNQENIPTGRLLTVDDSSYSIKESVSIKKLLKDNPEGLDDCFVFNPKGDKSLMLYDPLSGRKLVAQTDRQAVVIYTATNPEIESMINGRPMSKNRGIAIEFQEIPDLVHHPEWGTIELKAGQKKTFITEYLFTTN

SEQ ID NO: 28 - protein, 442 aa, Eubacterium saburreum; identical to SEQ ID NO: 15

SEQ ID NO: 29 - protein, 437 aa, Piromyces sp. E2
MAKEYFPQIQKIKFEGKDSKNPLAFHYYDAEKEVMGKKMKDWLRFAMAWWHTLCAEGADQFGGGTKSFPWNEGTDAIEIAKQKVDAGFEIMQKLGIPYYCFHDVDLVSEGNSIEEYESNLKAVVAYLKEKQKETGIKLLWSTANVFGHKRYMNGASTNPDFDVVARAIVQIKNAIDAGIELGAENYVFWGGREGYMSLLNTDQKREKEHMATMLTMARDYARSKGFKGTFLIEPKPMEPTKHQYDVDTETAIGFLKAHNLDKDFKVNIEVNHATLAGHTFEHELACAVDAGMLGSIDANRGDYQNGWDTDQFPIDQYELVQAWMEIIRGGGFVTGGTNFDAKTRRNSTDLEDIIIAHVSGMDAMARALENAAKLLQESPYTKMKKERYASFDSGIGKDFEDGKLTLEQVYEYGKKNGEPKQTSGKQELYEAIVAMYQ

SEQ ID NO: 30 - protein, 437 aa, Orpinomyces sp. PC-2
MTKEYFPTIGKIRFEGKDSKNPMAFHYYDAEKEVMGKKMKDWLRFAMAWWHTLCADGADQFGVGTKSFPWNEGTDPIAIAKQKVDAGFEIMTKLGIEHYCFHDVDLVSEGNSIEEYESNLKQVVAYLKQKQQETGIKLLWSTANVFGNPRYMNGASTNPDFDVVARAIVQIKNAMDAGIELGAENYVFWGGREGYMSLLNTDQKREKEHMATMLTMARDYARSKGFKGTFLIEPKPMEPTKHQYDVDTETVIGFLRAHNLDKDFKVNIEVNHATLAGHTFEHELACAVDAGMLGSIDANRGDYQNGWDTDQFPIDQYELVQAWMEIIRGGGFVTGGTNFDAKTRRNSTDLEDIIIAHISGMDAMARALENAAKLLQESPYCNMKKERYASFDSGIGKDFEDGKLTLEQVYEYGKKNGEPKVTSGKQELYEAIVAMYQ

SEQ ID NO: 31 - protein, 438 aa, Clostridium phytofermentans
MKNYFPNVPEVKYEGPNSTNPFAFKYYDAERIVAGKTMKEHCRFALSWWHTLCAGGADPFGVTTMDRSYGNITDPMEFAKAKVDAGFELMTKLGIEYFCFHDADIAPEGENFEESKKNLFVIVDYIKEKMDQTGIKLLWGTANNFGHPRFMHGASTSCNADVFAYAAAKIKNALDATIKLGGKGYVFWGGREGYETLLNTDLGLELDNMARLMKMAVEYGRANGFDGDFYIEPKPKEPTKHQYDFDTATVLGFLRKYGLEKDFKMNIEANHATLAGHTFEHELALARVNGVFGSVDANQGDPNLGWDTDQFPTDVHSATLAMLEVLKAGGFTNGGLNFDAKVRRGSFEFDDIAYGYIAGMDTFALGLIKAAEIIEDGRIAKFVEDRYASYKTGIGKAIVDGTTSLEELEQYVLTHNEPVMQSGRQEVLESIVNNILFR

SEQ ID NO: 32 - protein, 438 aa, Ruminococcus flavefaciens
MEFFSNIGKIQYQGPKSTDPLSFKYYNPEEVINGKTMREHLKFALSWWHTMGGDGTDMFGCGTTDKTWGQSDPAARAKAKVDAAFEIMDKLSIDYYCFHDRDLSPEYGSLKATNDQLDIVTDYIKEKQGDKFKCLWGTAKCFDHPRFMHGAGTSPSADVFAFSAAQIKKALESTVKLGGNGYVFWGGREGYETLLNTNMGLELDNMARLMKMAVEYGRSIGFKGDFYIEPKPKEPTKHQYDFDTATVLGFLRKYGLDKDFKMNIEANHATLAQHTFQHELRVARDNGVFGSIDANQGDVLLGWDTDQFPTNIYDTTMCMYEVIKAGGFTNGGLNFDAKARRGSFTPEDIFYSYIAGMDAFALGFRAALKLIEDGRIDKFVADRYASWNTGIGADIIAGKADFASLEKYALEKGEVTASLSSGRQEMLESIVNNVLFSL

SEQ ID NO: 33 - protein, 438 aa, Bacteroides uniformis
MATKEYFPGIGKIKFEGKESKNPMAFRYYDADKVIMGKKMSEWLKFAMAWWHTLCAEGGDQFGGGTKKFPWNGEADKVQAAKNKMDAGFEFMQKMGIEYYCFHDVDLCEEAETIEEYEANLKEIVAYAKQKQAETGIKLLWGTANVFGHARYMNGAATNPDFDVVARAAIQIKNAIDATIELGGSNYVFWGGREGYMSLLNTDQKREKEHLAQMLTIARDYARARGFKGTFLIEPKPMEPTKHQYDVDTETVIGFLKAHNLDKDFKVNIEVNHATLAGHTFEHELAVAVDNGMLGSIDANRGDYQNGWDTDQFPIDNFELTQAMMQIIRNGGFGNGGTNFDAKTRRNSTDLEDIFIAHIAGMDVMARALESAAKLLEESPYKKMLADRYASFDSGKGKEFEDGKLTLEDLVAYAKANGEPKQTSGKQELYEAIVNMYC

SEQ ID NO: 34 - protein, 439 aa, Clostridium cellulolyticum
MSEVFSGISNIKFEGSGSDNPLAFKYYDPKAVIGGKTMEEHLRFAVAYWHTFAAPGADMFGAGSYVRPWNTMSDPLEIAKYKVEANFEFIEKLGAPFFAFHDRDIAPEGDTLAETNKNLDTIVSVIKDRMKSSPVKLLWGTTNAFGNPRFMHGASTSPNADIFAYAAAQVKKAMEITKELGGENYVFWGGREGYETLLNTDMKLELDNLARFLKMAVDYAKEIGFDGQFLIEPKPKEPTKHQYDFDTATVIGFLKTYGLDPYFKMNIEANHATLAGHTFQHELAMCRINDMLGSIDANQGDVMLGWDTDQFPTNLYDATLAMVEVLKAGGLKKGGLNFDSKVRRGSFEPSDLFYGHIAGMDTFAKGLIIANKIVEDGKFDAFVADRYSSYTNGIGKDIVEGKVGFKELEQYALTAKIQNKSGRQEMLEALLNQYILETK

SEQ ID NO: 35 - protein, 444 aa, Thermotoga maritima
MAEFFPEIPKIQFEGKESTNPLAFRFYDPNEVIDGKPLKDHLKFSVAFWHTFVNEGRDPFGDPTAERPWNRFSDPMDKAFARVDALFEFCEKLNIEYFCFHDRDIAPEGKTLRETNKILDKVVERIKERMKDSNVKLLWGTANLFSHPRYMHGAATTCSADVFAYAAAQVKKALEITKELGGEGYVFWGGREGYETLLNTDLGLELENLARFLRMAVEYAKKIGFTGQFLIEPKPKEPTKHQYDFDVATAYAFLKNHGLDEYFKFNIEANHATLAGHTFQHELRMARILGKLGSIDANQGDLLLGWDTDQFPTNIYDTTLAMYEVIKAGGFTKGGLNFDAKVRRASYKVEDLFIGHIAGMDTFALGFKIAYKLAKDGVFDKFIEEKYRSFKEGIGKEIVEGKTDFEKLEEYIIDKEDIELPSGKQEYLESLLNSYIVKTIAELR

SEQ ID NO: 36 - protein, 441 aa, Geobacillus stearothermophilus
MPYFDNISTIAYEGPASKNPLAFKFYNPEEKVGDKTMEEHLRFSVAYWHTFTGDGSDPFGAGNMIRPWNKYSGMDLAKARVEAAFEFFEKLNIPFFCFHDVDIAPEGETLKETYKNLDIIVDMIEEYMKTSKTKLLWNTANLFTHPRFVHGAATSCNADVFAYAAAKVKKGLEIAKRLGAENYVFWGGREGYETLLNTDMKLELDNLARFLHMAVDYAKEIGFDGQFLIEPKPKEPTKHQYDFDVATALAFLQTYGLKDYFKFNIEANHATLAGHTFEHELRVARIHGMLGSVDANQGDMLLGWDTDEFPTDLYSTTLAMYEILKNGGLGRGGLNFDAKVRRGSFEPEDLFYAHIAGMDSFAVGLKVAHRLIEDRVFDEFIEERYKSYTEGIGREIVEGTADFHKLEAHALQLGEIQNQSGRQERLKTLLNQYLLEVCAAR

SEQ ID NO: 37 - protein, 438 aa, Bacteroides stercoris
MATKEYFPGIGKIKFEGKESKNPMAFRYYDAEKVIMGKKMKDWLKFSMAWWHTLCAEGGDQFGGGTKHFPWNGDADKLQAAKNKMDAGFEFMQKMGIEYYCFHDVDLCDEADTIEEYEANLKAIVAYAKQKQEETGIKLLWGTANVFGHARYMNGAATNPDFDVVARAAVQIKNAIDATIELGGSNYVFWGGREGYMSLLNTDQKREKEHLAQMLTIARDYARARGFKGTFLIEPKPMEPTKHQYDADTETVVGFLKAHGLDKDFKVNIEVNHATLAGHTFEHELAVAVDNGMLGSIDANRGDYQNGWDTDQFPIDNYELTQAMMQIIRNGGFGDGGTNFDAKTRRNSTDLEDIFIAHIAGMDVMARALESAAKLLEESPYKKMLADRYASFDSGKGKEFEEGKLTLEDVVAYAKANGEPKQTSGKQELYEAIVNMYC

SEQ ID NO: 38 - protein, 442 aa, Parabacteroides distasonis
MSYFKGEKEFFPGIGQIQFEGRESKNPLAFHYYDADKVVMGKTLKDHLRFAMAYWHTLCAEGGDQFGGGTKTFPWNDSTDAITRAKYKMDAAFEFMTKCNIPYYCFHDVDVVDEAPTLGEFEKRLQTMVEHAKEHQAATGKKLLWSTANVFGHKRYMNGAATNPYFPTVACAGTQIKNAIDACIALGGENYVFWGGREGYMSLLNTNMKREKDHLAMMLTMARDYGRKNGFKGTFLIEPKPMEPTKHQYDVDSETVIGFLRHYGLDKDFALNIEVNHATLAGHTFEHELQAAADAGMLCSIDANRGDYQNGWDTDQFPMDIYELAQAWLVILEGGGLTTGGTNFDAKTRRNSTDLEDIFIAHIGGMDAFARALMIAADILENSDYRKMRAERYASFDAGEGKAFEDGKLTLEDLRTIALRDGEPKQISGKQELYEMIVNLHI

SEQ ID NO: 39 - protein, 439 aa, Prevotella ruminicola
MAKEYFPFTGKIPFEGKDSKNVMAFHYYEPEKVVMGKKMKDWLKFAMAWWHTLGGASADQFGGQTRSYEWDKAADAVQRAKDKMDAGFEIMDKLGIEYFCFHDVDLVEEGETIAEYERRMKEITDYALVKMKEYPNIKLLWGTANVFGNKRYANGASTNPDFDVVARAIVQIKNAIDATIKLGGTNYVFWGGREGYMSLLNTDQKREKEHMATMLTMARDYARAKGFKGTFLIEPKPMEPSKHQYDVDTETVCGFLRAHGLDKDFKVNIEVNHATLAGHTFEHELACAVDNGMLGSIDANRGDAQNGWDTDQFPIDNFELTQAMLEIIRNGGLGNGGTNFDAKIRRNSTDLEDLFIAHISGMDAMARALMNAAAILEESELPKMKKERYASFDNGIGKDFEDGKLTLEQAYEYGKKVEEPKQTSGKQEKYETTVALYCK

SEQ ID NO: 40 - protein, 436 aa, Agrobacterium tumefaciens
MSTGFFGDITKIKYEGPDSTNPLAFRHYNPDEIVAGKRMEDHLRFAVAYWHTFTWPGGDPFGGQTFQRPWFEDTMQAAKLKADVAFEFFSLLGSPFYCFHDADVRPEGKNFAENTKNLNEIVDYFAEKQAQTGVKLLWGTANLFSNRRFMSGAATNPDPDVFAFSAATVKTCLDATKKLGGANYVLWGGREGYETLLNTDLSRELDQMGRFLNLVVEYKYKIGFEGTILIEPKPQEPTKHQYDYDVATVYAFLQKNGLEKEVKVNIEQGHAILAGHSFEHELALANAFGIFGSIDMNRNDYQSGWDTDQFPNNVPEMALAYYHVLAGGGFKNGGTNFDAKLRRQSLDPQDLLIGHIGGMDCCARGLKAAAKMIEDGALSKPLSERYAKWDSAEAQKMLRGELKLDDIAALVEREDINPEPKSGRQEYLENVVNRYV

SEQ ID NO: 41 - protein, 439 aa, Clostridium cellulovorans
MREYFANVPKIKYEGKDSKNPLAFKYYNPDEVVGGKTMKEHLRFTLSYWHTLTGAGSDPFGVGTMLRPWDCAEDEMELAKMRMEANFELMDKLGIEYFAFHDRDIAPEGKTLADTNEKLDEIVAYCKELMQKHGKKLLWGTANMFGNPRFVHGAATTCNADVFAYAAAQTKKAMDVTKELGGENYVFWGGREGYETLLNTDLGLEQDNLARFFQMAVDYAKKIGFTGQFLIEPKPKEPTKHQYDFDVATVLGFLRKYNLEKYFKMNIEANHATLAQHTFQHEVAVARVNGVLGSLDVNQGDPNLGWDTDQFPTNIYDATMVMYEVLKNGGIAPGGLNFDAKTRRASFEPEDLFLSYIAGMDTMAKGLRVAYSLLDDAVLENNTSERYKTFSEGIGKDIVEGKVDFESLEKYALENSVISNKSGRQEYLESVVNQYIFND

SEQ ID NO: 42 - protein, 440 aa, Burkholderia cenocepacia
MSYFEHIPAIRYEGPQSDNPLAYHHYDPDKRVLGKTLAEHLRIAVCYWHTFVWPGHDIFGQGAFQRPWQQPGDALERARQKADAAFEFFTKLGTPFYTFHDTDVAPEGDSLRDYAANFARMVDYLGERQQASGVRLLWGTANLFSHPRFAAGAATNPNPDVFAWAATQVCHALDATHRLGGENYVLWGGREGYETLLNTDLKRERDQFARFLSMVVEHKHRIGFKGALLIEPKPQEPTKHQYDYDVATVHGFLVQYGLQNEIRVNIEANHATLAGHSFHHEIANAFALGVFGSVDANRGDPQNGWDTDQFPNSVEELTLAFYEILRHGGFTTGGMNFDAKVRRQSIDPEDLFYGHVGAIDVLALALERAAVLVENDRLDALRRQRYAQWDDAFGRKILSGGYTLESLAADALARGVNPRHASGAQERLENIVNQAIYGLR

SEQ ID NO: 43 - protein, 439 aa, Lactococcus lactis
MAYFNDIAPIKYEGTKTKNMFAFRHYNPEEVVAGKTMEEQLHFALAFWHTITMDGSDPFGGATMERPWDLEGGSELDRAHRRVDAFFEIAEKLGVKYYCFHDIDIAPTGNSLKEFYANLDEITDHLLEKQKATGIKLLWNTANMFSNPRYMNGVSTSNRAEVFAYGAAQVKKGLELSKKLGGENYVFWGGREGYESLLNTDMGLEMDHMAKFFHLAIDYAKSINHLPIFLIEPKPKEPMTHQYDFDSATALAFLQKYDLDKYFKLNLETNHAWLAGHTFEHELNTARTFNALGSIDANQGNYLLGWDTDEFPTLVIDITLAMHQILLNGGLGKGGINFDAKVRRTSFKAEDLILAHIAGMDTYARALKGAAAIIEDKFLSDIVDERYSSYRNTEVGQSIENGTATFESLAAFALEYGDDIELDSNHLEYIKSVLNDYLV

SEQ ID NO: 44 - protein, 438 aa, Thermoanaerobacter thermohydrosulfuricus
MEYFKNVPQIKYEGPKSNNPYAFKFYNPDEIIDGKPLKEHLRFSVAYWHTFTANGTDPFGAPTMQRPWDHFTDPMDIAKARVEAAFELFEKLDVPFFCFHDRDIAPEGETLRETNKNLDTIVAMIKDYLKTSKTKVLWGTANLFSNPRFVHGAATSCNADVFAYAAAQVKKALEITKELGGQNYVFWGGREGYETLLNTDMELELDNLARFLHMAVEYAQEIGFEGQFLIEPKPKEPTKHQYDFDAASVHAFLKKYDLDKYFKLNIEANHATLAGHDFQHELRYARINNMLGSIDANMGDMLLGWDTDQYPTDIRMTTLAMYEVIKMGGFNKGGLNFDAKVRRASFEPEDLFLGHIAGMDAFAKGFKVAYKLVKDGVFDRFIEERYKSYREGIGAEIVSGKANFKTLEEYALNNPKIENKSGKQELLESILNQYLFSE

SEQ ID NO: 45 - protein, 439 aa, Reticulitermes speratus
MSQIFKDIPVIKYEGPASKNPLSFKYYDANKVIDGKPMKEHLRYAMAWWHNLCATGQDMFGPGTADKSFGSKTVGTMEHAHAKVDAGFEFMSKLGVEYFCFHDADLVPEADTLSETNKRLDEIAEHIVAKQKATGIKCLWGTANLFSNPRFLNGSGSSNSADVYAYAAAQIKKALDLTVKFGGVGYVFWGGREGYETLLNTDVKFEQENIANLMHLAVTYGRSIGFKGDFYIEPKPKEPTKHQYDFDAATTIGFIRQYGLEKDFKLNIEANHATLAGHTFQHDLRISAINGMLGSVDANTGDPLLGWDTDEFPYSVYDTTLAMYEIIKAGGLTGGLNFDSKVRRPSYTHEDLFYGFILGMDSFALGLIKAKALIADGRLDSFVKDRYASYGSGIGAKIRDHSATLEELAAYALAKDTVALPGSGRQEYLESIINQILFQ

SEQ ID NO: 46 - protein, 438 aa, uncultured bacterium
  uncultured bacteria from cow rumen
MSEIFANIPVIPYEGPQSKNPLAFKFYDADKVILGKKMSEHLPFAMAWWHNLCAGGTDMFGRDTADKSFGAEKGTMAHARAKVDAGFEFMKKVGVKYFCFHDVDLVPEADDIKETNRRLDEISDYILEKMKGTDIKCLWGTANMFGNPRYMNGAGSTNSADVFCFAAAQIKKALDLTVKLGGRGYVFWGGREGYETLLNTDMKFEQENIARLMHLAVDYGRSIGFTGDFYIEPKPKEPMKHQYDFDAATAIGFLRQYGLDKDFKMNIEANHATLAGHTFQHDLRISAINGMLGSIDANQGDLLLGWDTDEFPFNVYEATLCMYEVLKAGGLTGGFNFDSKTRRPSYTLEDMFHAYILGMDTFALGLIKAAALIEDGRLDQFVADRYASYKTGIGAKIRSGETTLAELAAYADKLGAPALPSSGRQEYLESIVNSILFG

SEQ ID NO: 47 - protein, 438 aa, uncultured bacterium
  uncultured bacteria from cow rumen
MAEIFKGIPEIRYEGPNSTNPLSFKYYDPDKVILGKPMKEHLPFAMAWWHNLGAAGTDMFGRDTADKSFGAEKGTMEHAKAKVDAGFEFMKKLGIRYFCFHDVDLVPEADDIKVTNARLDEISDYILEKMKGTDIKCLWGTANMFSNPRFMNGAGSTNSADVFCFAAAQVKKALDITVKLGGKGYVFWGGREGYETLLNTDVKFEQENIAKLMHLAVDYGRSIGFKGDFFIEPKPKEPMKHQYDFDAATAIGFVRQYGLDKDFKMNIEANHATLAGHTFQHELRISAINGMLGSIDANQGDMLLGWDTDEFPFNVYDTTLCMYEVLKNGGIPGGFNFDAKNRRPSYTAEDMFYGFILGMDSFALGLIKAAKLIEDGRIDKFVEERYASYKDGIGKKIRDGETTLAELAAYADQLGAPKLPGSGRQEDLESVFNQVLFG

SEQ ID NO: 48 - protein, 442 aa, Lachnoanaerobaculum
MKEFFPSISPIKFEGSESKNPLSFKYYDAKRVIMGKTMEEHLSFAMAWWHNLCASGVDMFGQGTADKGFGENLGTMEHAKAKVDAGIEFMQKLGIKYYCFHDTDIVPEDQEDINVTNARLDEITDYILEKTKGTDIKCLWATCNMFSNPRFMNGAGSSNSADVFCFAAAQAKKGLENAVKLGAKGFVFWGGREGYETLLNTDMKLEEENIATLFTMCRDYGRSIGFKGDFYIEPKPKEPMKHQYDFDAATAIGFLRKYGLDKDFKMNIEANHATLAGHTFQHELRVSAINGMLGSVDANQGDTLLGWDTDQFPTNVYDTTLAMYEILKAGGLSGGLNFDSKNRRPSNTAEDMFYGFIAGMDTFALGLIKAAQIIEDGRIDEFVKERYSSYNSGIGEKIRNRSVTLVECAEYALKMKKPELPESGRQEYLETVVNNIFFNSKL

SEQ ID NO: 49 - protein, 442 aa, Lachnospiraceae bacterium oral taxon 500
MKEFFPGISPVKFEGSESKNPLSFKYYDAKRVIMGKTMEEHLSFAMAWWHNLCASGVDMFGQGTADKGFGESSGTMGHAKAKVDAGIEFMKKLGIKYYCFHDTDIVPEDQEDINVTNARLDEITDYILEKTKGSDIKCLWTTCNMFGNPRFMNGAGSSNSADVFCFAAAQAKKGLENAVKLGAKGFVFWGGREGYETLLNTDMKLEEENIATLFTMCRDYGRSIGFKGDFYIEPKPKEPMKHQYDFDAATAIGFLRKYGLDKDFKLNIEANHATLAGHTFQHELRVSAINGMLGSVDANQGDTLLGWDTDQFPTNIYDTTFAMYEILKAGGLSGGLNFDSKNRRPSNTAEDMFYGFIAGMDTFALGLIKAAQIIEDGRIDEFIKERYSSYSTGIGEKIRNKSVTLEECAEYAAKLKKPELPESGRQEYLETVVNNILFNSKL

SEQ ID NO: 50 - protein, 439 aa, Lachnospiraceae bacterium oral taxon 082
MKEFFPGISPVKFEGKDSKNPLSFKYYDAKRVIMGKTMEEHLSFAMAWWHNLCACGVDMFGQGTIDKSFGALPGTMEHAKAKVDAGIEFMQKLGIKYYCFHDTDIVPEDQEDINVTNARLDEITDYILEKTKGTDIKCLWTTCNMFSNPRFMNGAGSSNSADVFCFAAAQAKKGLENAVKLGAKGFVFWGGREGYETLLNTDMKLEEENIATLFTMCRDYGRSIGFMGDFYIEPKPKEPMKHQYDFDAATAIGFLRKYGLEKDFKMNIEANHATLAGHTFQHELRVCAVNGMIGSVDANQGDTLLGWDTDQFPTNVYDTTLAMYEILKAGGLRGGLNFDSKNRRPSNTADDMFYGFIAGMDAFALGLIKAAEIIEDGRIDEFVKERYSSYNSGIGEKIRNRAVTLVECAEYAAKLKKPELPDSGKQEYLESVVNNILFG

SEQ ID NO: 51 - protein, 443 aa, uncultured bacterium
MSVVLGDKEYFPGVGKIAYEGPESDNPLSFKWYDENRVVAGKTLKDHFKFAVCYWHTFCGAGHDSFGPGPFVFPWGAGSDALSRAKMKADAAFEFITKLGVPYYCFHDIDLIEEGSSRAETAKRVMDIVEYAKQKQAASGVKLLWGTANLFSNPRYINGASTNPDFAVVAHAGAQLKDALDATIALGGENYVFWGGREGYMSPLNTDMKREVERFARFLTMARDYARGQGFKGVFFIEPKPMEPSKHQYDFDCATVIGFLRQYGLDKDFKLNIETNHATLAGHTMEHEMQVAADAGMLGSIDANRGDYQNAWDTDQFPNNINETTEMMLVLLRSGGFQGGGVNFDAKRRRNSTDPNDTFHGHIGGMDTFARSLIIAGDILEKSPIEKMRKERYASFDAGKGAEFEAGKLSLVQLAELGNKGGEPTQKSGRQELYENIMNRWIR

SEQ ID NO: 52 - protein, 442 aa, uncultured bacterium
MKLTVGDKEYFKGIKPIKFEGKDSDNPLAFKYYNPSQKVGKKTMEEHFRFAIAYWHTFCGTGGDPFGPGTKTFPWLQNSDAVQRAYDKMDAAFEFITKIGAPFYCFHDYDLVDEGPTLKESESRLQKVVDYAKKKQKASGVKLLWGTANLFSHPRYMNGAATNPDFDVVCYAASQVKNALDATIALGGANYVFWGGREGYMSLLNTNMKREQEHMAKFLHMAKDYARANGFKGTFFIEPKPMEPSKHQYDFDSATVIGFLRQFDLLGDFKLNIEVNHATLAHHTFQHELQVAADAGALGSIDANRGDYQNGWDTDQFPNNLYELAESMLVILEAGGFKSGGVNFDAKTRRNSTDLVDIFHAHIGGMDTFARSLLIAQAVLDNGEYTKIRKDRYSSFDSGKGKQFDQGKLSLEDLRNLAHKAGEPKQLSGKQEYIENLISRFI

SEQ ID NO: 53 - protein, 387 aa, Thermus thermophilus
MYEPKPEHRFTFGLWTVGNVGRDPFGDAVRERLDPVYVVHKLAELGAYGVNLHDEDLIPRGTPPQERDQIVRRFKKALDETGLKVPMVTANLFSDPAFKDGAFTSPDPWVRAYALRKSLETMDLGAELGAEIYVVWPGREGAEVEATGKARKVWDWVREALNFMAAYAEDQGYGYRFALEPKPNEPRGDIYFATVGSMLAFIHTLDRPERFGLNPEFAHETMAGLNFVHAVAQALDAGKLFHIDLNDQRMSRFDQDLRFGSENLKAAFFLVDLLESSGYQGPRHFDAHALRTEDEEGVWAFARGCMRTYLILKERAEAFREDPEVKELLAAYYQEDPAALALLGPYSREKAEALKRAELPLEAKRRRGYALERLDQLAVEYLLGVRG

SEQ ID NO: 54 - protein, 440 aa, Escherichia coli
MQAYFDQLDRVRYEGSKSSNPLAFRHYNPDELVLGKRMEEHLRFAACYWHTFCWNGADMFGVGAFNRPWQQPGEALALAKRKADVAFEFFHKLHVPFYCFHDVDVSPEGASLKEYINNFAQMVDVLAGKQEESGVKLLWGTANCFTNPRYGAGAATNPDPEVFSWAATQVVTAMEATHKLGGENYVLWGGREGYETLLNTDLRQEREQLGRFMQMVVEHKHKIGFQGTLLIEPKPQEPTKHQYDYDAATVYGFLKQFGLEKEIKLNIEANHATLAGHSFHHEIATAIALGLFGSVDANRGDAQLGWDTDQFPNSVEENALVMYEILKAGGFTTGGLNFDAKVRRQSTDKYDLFYGHIGAMDTMALALKIAARMIEDGELDKRIAQRYSGWNSELGQQILKGQMSLADLAKYAQEHHLSPVHQSGRQEQLENLVNHYLFDK

SEQ ID NO: 55 - protein, 600 aa, Saccharomyces cerevisiae
MLCSVIQRQTREVSNTMSLDSYYLGFDLSTQQLKCLAINQDLKIVHSETVEFEKDLPHYHTKKGVYIHGDTIECPVAMWLEALDLVLSKYREAKFPLNKVMAVSGSCQQHGSVYWSSQAESLLEQLNKKPEKDLLHYVSSVAFARQTAPNWQDHSTAKQCQEFEECIGGPEKMAQLTGSRAHFRFTGPQILKIAQLEPEAYEKTKTISLVSNFLTSILVGHLVELEEADACGMNLYDIRERKFSDELLHLIDSSSKDKTIRQKLMRAPMKNLIAGTICKYFIEKYGFNTNCKVSPMTGDNLATICSLPLRKNDVLVSLGTSTTVLLVTDKYHPSPNYHLFIHPTLPNHYMGMICYCNGSLARERIRDELNKERENNYEKTNDWTLFNQAVLDDSESSENELGVYFPLGEIVPSVKAINKRVIFNPKTGMIEREVAKFKDKRHDAKNIVESQALSCRVRISPLLSDSNASSQQRLNEDTIVKFDYDESPLRDYLNKRPERTFFVGGASKNDAIVKKFAQVIGATKGNFRLETPNSCALGGCYKAMWSLLYDSNKIAVPFDKFLNDNFPWHVMESISDVDNENWDRYNSKIVPLSELEKTLI

SEQ ID NO: 56 - protein, 623 aa, Scheffersomyces stipitis
MTTTPFDAPDKLFLGFDLSTQQLKIIVTDENLAALKTYNVEFDSINSSVQKGVIAINDEISKGAIISPVYMWLDALDHVFEDMKKDGFPFNKVVGISGSCQQHGSVYWSRTAEKVLSELDAESSLSSQMRSAFTFKHAPNWQDHSTGKELEEFERVIGADALADISGSRAHYRFTGLQIRKLSTRFKPEKYNRTARISLVSSFVASVLLGRITSIEEADACGMNLYDIEKREFNEELLAIAAGVHPELDGVEQDGEIYRAGINELKRKLGPVKPITYESEGDIASYFVTRYGFNPDCKIYSFTGDNLATIISLPLAPNDALISLGTSTTVLIITKNYAPSSQYHLFKHPTMPDHYMGMICYCNGSLAREKVRDEVNEKFNVEDKKSWDKFNEILDKSTDFNNKLGIYFPLGEIVPNAAAQIKRSVLNSKNEIVDVELGDKNWQPEDDVSSIVESQTLSCRLRTGPMLSKSGDSSASSSASPQPEGDGTDLHKVYQDLVKKFGDLYTDGKKQTFESLTARPNRCYYVGGASNNGSIIRKMGSILAPVNGNYKVDIPNACALGGAYKASWSYECEAKKEWIGYDQYINRLFEVSDEMNSFEVKDKWLEYANGVGMLAKMESELKH

SEQ ID NO: 57 - protein, 575 aa, Trichoderma reesei
MSEEKGPLYLGFDLSTQQLKAIVVNSNLKSIAEAKVDFDQDFGPQYGIQKGVHVRESTGEVFAPVALWLESLDLVLSRLSKAMHPLPMSRIRGVSGSGQQHGAVFWNASAEELLGGLDAAKGSLVEQLRGALAHEFAPNWQDHSTQEELVAFDAELGDREKLAEVTGSGAHHRFTGLQIMRIRRVLPQVYANAKRISLVSSWLASVLMGSIAPLDVSDVCGMNLWDIPNQAWSEKLLALSGGGGLDGAANLRRKLGEPRMDGGGSMGSISRYYVSKYGFSPECQITPFTGDNPATILALPLRPLDAIVSLGTSTTFLMNTPAYKPDGSYHFFNHPTTPGNYMFMLCYKNGGLAREKVRDTLPKPEGGATGWETFNEAIMATKPLGIESDGDRAKLGLYFYLRETVPNIRAGTWRFTCRQDGSDLQEAREAWPKEADARAIVESQALSMRLRSQKLVHSPRDGLPAQPRRIYVVGGGSLNPAITRVLGEVLGGADGVYKLDVGGNACALGGAYKALWALERKDGETFDDLIGGRWTEEGSIDKVDVGYREGTYERYGKVLGAFEEMERRLLAEEEH

SEQ ID NO: 58 - protein, 335 aa, Saccharomyces cerevisiae
MSEPAQKKQKVANNSLEQLKASGTVVVADTGDFGSIAKFQPQDSTTNPSLILAAAKQPTYAKLIDVAVEYGKKHGKTTEEQVENAVDRLLVEFGKEILKIVPGRVSTEVDARLSFDTQATIEKARHIIKLFEQEGVSKERVLIKIASTWEGIQAAKELEEKDGIHCNLTLLFSFVQAVACAEAQVTLISPFVGRILDWYKSSTGKDYKGEADPGVISVKKIYNYYKKYGYKTIVMGASFRSTDEIKNLAGVDYLTISPALLDKLMNSTEPFPRVLDPVSAKKEAGDKISYISDESKFRFDLNEDAMATEKLSEGIRKFSADIVTLFDLIEKKVTA

SEQ ID NO: 59 - protein, 333 aa, Saccharomyces cerevisiae
MSEPSEKKQKVATSSLEQLKKAGTHVVADSGDFEAISKYEPQDSTTNPSLILAASKLEKYARFIDAAVEYGRKHGKTDHEKIENAMDKILVEFGTQILKVVPGRVSTEVDARLSFDKKATVKKALHIIKLYKDAGVPKERVLIKIASTWEGIQAARELEVKHGIHCNMTLLFSFTQAVACAEANVTLISPFVGRIMDFYKALSGKDYTAETDPGVLSVKKIYSYYKRHGYATEVMAASFRNLDELKALAGIDNMTLPLNLLEQLYESTDPIENKLNSESAKEEGVEKVSFINDEPHFRYVLNEDQMATEKLSDGIRKFSADIEALYKLVEEKM

SEQ ID NO: 60 - protein, 323 aa, Scheffersomyces stipitis
MSSNSLEQLKATGTVIVTDTGEFDSIAKYTPQDATTNPSLILAAAKKPEYAKVIDVAIEYAKDKGSSKKEKAEIALDRLLIEFGKNILAIVPGRVSTEVDARLSFDKEATIKKALELIALYESQGISKDRILIKIASTWEGIQAARELEAKHGIHCNLTLLFSFVQAVACAEAKVTLISPFVGRILDWYKASTGKTYEGDEDPGVISVRAIYNYYKKYGYKTIVMGASFRNTGEIKALAGCDYLTVAPKLLEELLNSTEPVPQVLDAASASATDVEKVSYVDDEATFRYLFNEDAMATEKLAQGIRAFGKDAVTLLEQLEARF

SEQ ID NO: 61 - protein, 680 aa, Saccharomyces cerevisiae
MTQFTDIDKLAVSTIRILAVDTVSKANSGHPGAPLGMAPAAHVLWSQMRMNPTNPDWINRDRFVLSNGHAVALLYSMLHLTGYDLSIEDLKQFRQLGSRTPGHPEFELPGVEVTTGPLGQGISNAVGMAMAQANLAATYNKPGFTLSDNYTYVFLGDGCLQEGISSEASSLAGHLKLGNLIAIYDDNKITIDGATSISFDEDVAKRYEAYGWEVLYVENGNEDLAGIAKAIAQAKLSKDKPTLIKMTTTIGYGSLHAGSHSVHGAPLKADDVKQLKSKFGFNPDKSFVVPQEVYDHYQKTILKPGVEANNKWNKLFSEYQKKFPELGAELARRLSGQLPANWESKLPTYTAKDSAVATRKLSETVLEDVYNQLPELIGGSADLTPSNLTRWKEALDFQPPSSGSGNYSGRYIRYGIREHAMGAIMNGISAFGANYKPYGGTFLNFVSYAAGAVRLSALSGHPVIWVATHDSIGVGEDGPTHQPIETLAHFRSLPNIQVWRPADGNEVSAAYKNSLESKHTPSIIALSRQNLPQLEGSSIESASKGGYVLQDVANPDIILVATGSEVSLSVEAAKTLAAKNIKARVVSLPDFFTFDKQPLEYRLSVLPDNVPIMSVEVLATTCWGKYAHQSFGIDRFGASGKAPEVFKFFGFTPEGVAERAQKTIAFYKGDKLISPLKKAF

SEQ ID NO: 62 - protein, 681 aa, Saccharomyces cerevisiae
MAQFSDIDKLAVSTLRLLSVDQVESAQSGHPGAPLGLAPVAHVIFKQLRCNPNNEHWINRDRFVLSNGHSCALLYSMLHLLGYDYSIEDLRQFRQVNSRTPGHPEFHSAGVEITSGPLGQGISNAVGMAIAQANFAATYNEDGFPISDSYTFAIVGDGCLQEGVSSETSSLAGHLQLGNLITFYDSNSISIDGKTSYSFDEDVLKRYEAYGWEVMEVDKGDDDMESISSALEKAKLSKDKPTIIKVTTTIGFGSLQQGTAGVHGSALKADDVKQLKKRWGFDPNKSFVVPQEVYDYYKKTVVEPGQKLNEEWDRMFEEYKTKFPEKGKELQRRLNGELPEGWEKHLPKFTPDDDALATRKTSQQVLTNMVQVLPELIGGSADLTPSNLTRWEGAVDFQPPITQLGNYAGRYIRYGVREHGMGAIMNGISAFGANYKPYGGTFLNFVSYAAGAVRLAALSGNPVIWVATHDSIGLGEDGPTHQPIETLAHLRAIPNMHVWRPADGNETSAAYYSAIKSGRTPSVVALSRQNLPQLEHSSFEKALKGGYVIHDVENPDIILVSTGSEVSISIDAAKKLYDTKKIKARVVSLPDFYTFDRQSEEYRFSVLPDGVPIMSFEVLATSSWGKYAHQSFGLDEFGRSGKGPEIYKLFDFTADGVASRAEKTINYYKGKQLLSPMGRAF

SEQ ID NO: 63 - protein, 677 aa, Scheffersomyces stipitis
MSSVDQKAISTIRLLAVDAVAAANSGHPGAPLGLAPAAHAVFKKMRFNPKDTKWINRDRFVLSNGHACALLYSMLVLYGYDLTVEDLKKFRQLGSKTPGHPENTDVPGAEVTTGPLGQGICNGVGIALAQAQFAATYNKPDFPISDSYTYVFLGDGCLMEGVSSEASSLAGHLQLGNLIAFWDDNKISIDGSTEVAFTEDVIARYKSYGWHIVEVSDADTDITAIAAAIDEAKKVTNKPTLVRLTTTIGFGSLAQGTHGVHGAPLKADDIKQLKTKWGFNPEESFAVPAEVTASYNEHVAENQKIQQQWNELFAAYKQKYPELGAELQRRLDGKLPENWDKALPVYTPADAAVATRKLSEIVLSKIIPEVPEIIGGSADLTPSNLTKAKGTVDFQPAATGLGDYSGRYIRYGVREHAMGAIMNGIAAFGANYKNYGGTFLNFVSYAAGAVRLSALSEFPITWVATHDSIGLGEDGPTHQPIETLAHFRATPNISVWRPADGNETSAAYKSAIESTHTPHILALTRQNLPQLEGSSIEKASKGGYTLVQQDKADIIIVATGSEVSLAVDALKVLEGQGIKAGVVSLPDQLTFDKQSEEYKLSVLPDGVPILSVEVMSTFGWSKYSHQQFGLNRFGASGKAPEIFKLFEFTPEGVAERAAKTVAFYKGKDVVSPLRSAF

SEQ ID NO: 64 - protein, 348 aa, Saccharomyces cerevisiae
MSIPETQKGVIFYESHGKLEYKDIPVPKPKANELLINVKYSGVCHTDLHAWHGDWPLPVKLPLVGGHEGAGVVVGMGENVKGWKIGDYAGIKWLNGSCMACEYCELGNESNCPHADLSGYTHDGSFQQYATADAVQAAHIPQGTDLAQVAPILCAGITVYKALKSANLMAGHWVAISGAAGGLGSLAVQYAKAMGYRVLGIDGGEGKEELFRSIGGEVFIDFTKEKDIVGAVLKATDGGAHGVINVSVSEAAIEASTRYVRANGTTVLVGMPAGAKCCSDVFNQVVKSISIVGSYVGNRADTREALDFFARGLVKSPIKVVGLSTLPEIYEKMEKGQIVGRYVVDTSK

SEQ ID NO: 65 - protein, 511 aa, Arthrobacter aurescens
  -
MPSATSNPANNTSLEQYEVWFLTGSQHLYGEDVLKQVAAQSQEIANALNANSNVPVKLVWKPVLTDSDAIRRTALEANADDSVIGVTAWMHTFSPAKMWIQGLDALRKPLLHLHTQANRDLPWADIDFDFMNLNQAAHGDREFGYIQSRLGVPRKTVVGHVSNPEVARQVGAWQRASAGWAAVRTLKLTRFGDNMRNVAVTEGDKTEAELRFGVSVNTWSVNELADAVHGAAESDVDSLVAEYERLYEVVPELKKGGARHESLRYSAKIELGLRSFLEANGSAAFTTSFEDLGALRQLPGMAVQRLMADGYGFGAEGDWKTAILVRAAKVMGGDLPGGASLMEDYTYHLEPGSEKILGAHMLEVCPSLTAKKPRVEIHPLGIGGKEDPVRMVFDTDAGPGVVVALSDMRDRFRLVANVVDVVDLDQPLPNLPVARALWEPKPNFATSAAAWLTAGAAHHTVLSTQVGLDVFEDFAEIAKTELLTIDEDTTIKQFKKELNWNAAYYKLAGGL

SEQ ID NO: 66 - protein, 505 aa, Clavibacter michiganensis
  -
MSRITTSLDHYEVWFLTGSQNLYGEETLQQVAEQSQEIARQLEEASDIPVRVVWKPVLKDSDSIRRMALEANASDGTIGLIAWMHTFSPAKMWIQGLDALQKPFLHLHTQANVALPWSSIDMDFMNLNQAAHGDREFGYIQSRLGVVRKTVVGHVSTESVRASIGTWMRAAAGWAAVHELKVARFGDNMRNVAVTEGDKTEAELKFGVSVNTWGVNDLVARVDAATDAEIDALVDEYETLYDIQPELRRGGERHESLRYGAAIELGLRSFLEEGGFGAFTTSFEDLGGLRQLPGLAVQRLMAEGYGFGAEGDWKTAVLIRAAKVMGSGLPGGASLMEDYTYHLVPGEEKILGAHMLEICPTLTTGRPSLEIHPLGIGGREDPVRLVFDTDPGPAVVVAMSDMRDRFRIVANVVEVVPLDEPLPNLPVARAVWKPAPDLATSAAAWLTAGAAHHTVMSTQVGVEVFEDFAEIARTELLVIDEDTTLKGFTKEVRWNQAYHRLAQGL

SEQ ID NO: 67 - protein, 502 aa, Gramella forsetii
  -
MTNFENKEVWFITGSQHLYGEETLRQVANNSKEIVEGLNGSDNVPVKLIHQDTVKSSDEITKVMLDANNSSSCIGVILWMHTFSPAKMWIKGLSIIKKPICHFHTQFNAEIPWSKIDMDFMNLNQSAHGDREFGFIMSRMRKKRKVIVGHWKTEVTQKKVGNWQRVALGWDELQHIKVARIGDNMRQVAVTEGDKVAAQIKFGVEVNAYDSSDVTQHIDKVSDDEVNSLLKKYEKDYDLTDALKDGGDQRQSLVDAAKIELGLRAFLEEGGFMAFTDTFENLGALKQLPGLAVQRLMADGYGFGAEGDWKTAALLRAMKVMAQGMEGGTSFMEDYTNHFTEGKDYVLGSHMLEICPSIADSKPTCEVHPLGIGGKEDPVRLVFNSPKGKALNASLVDMGTRFRLIVNEVEAVEPEADLPNLPVARVLWDPKPDMDTAVTAWILAGGAHHTVYTQALSTEFLEDFADIAGIELLVIDDNTSVRQFKDTLNANEAYYHLFQHGM

SEQ ID NO: 68 - protein, 474 aa, Lactobacillus plantarum subsp. plantarum ATCC 14917
  -
MLSVPDYEFWFVTGSQHLYGEEQLKSVAKDAQDIADKLNASGKLPYKVVFKDVMTTAESITNFMKEVNYNDKVAGVITWMHTFSPAKNWIRGTELLQKPLLHLATQYLNNIPYADIDFDYMNLNQSAHGDREYAYINARLQKHNKIVYGYWGDEDVQEQIARWEDVAVAYNESFKVKVARFGDTMRNVAVTEGDKVEAQIKMGWTVDYYGIGDLVEEINKVSDADVDKEYADLESRYEMVQGDNDADTYKHSVRVQLAQYLGIKRFLERGGYTAFTTNFEDLWGMEQLPGLASQLLIRDGYGFGAEGDWKTAALGRVMKIMSHNKQTAFMEDYTLDLRHGHEAILGSHMLEVDPSIASDKPRVEVHPLDIGGKDDPARLVFTGSEGEAIDVTVADFRDGFKMISYAVDANKPEAETPNLPVAKQLWTPKMGLKKGALEWMQAGGGHHTMLSFSLTEEQMEDYATMVGMTKAFLK

SEQ ID NO: 69 - protein, 496 aa, Bacillus subtilis
  -
MLQTKDYEFWFVTGSQHLYGEETLELVDQHAKSICEGLSGISSRYKITHKPVVTSPETIRELLREAEYSETCAGIITWMHTFSPAKMWIEGLSSYQKPLMHLHTQYNRDIPWGTIDMDFMNSNQSAHGDREYGYINSRMGLSRKVIAGYWDDEEVKKEMSQWMDTAAALNESRHIKVARFGDNMRHVAVTDGDKVGAHIQFGWQVDGYGIGDLVEVMDRITDDEVDTLYAEYDRLYVISEETKRDEAKVASIKEQAKIELGLTAFLEQGGYTAFTTSFEVLHGMKQLPGLAVQRLMEKGYGFAGEGDWKTAALVRMMKIMAKGKRTSFMEDYTYHFEPGNEMILGSHMLEVCPTVALDQPKIEVHSLSIGGKEDPARLVFNGISGSAIQASIVDIGGRFRLVLNEVNGQEIEKDMPNLPVARVLWKPEPSLKTAAEAWILAGGAHHTCLSYELTAEQMLDWAEMAGIESVLISRDTTIHKLKHELKWNEALYRLQK

SEQ ID NO: 70 - protein, 493 aa, Bacillus licheniformis
  -
MIQAKTHVFWFVTGSQHLYGEEAVQEVEEHSKMICNGLNDGDLRFQVEYKAVATSLDGVRKLFEEANRDEECAGIITWMHTFSPAKMWIPGLSELNKPLLHFHTQFNRDIPWDKIDMDFMNINQSAHGDREYGFIGARLGIPRKVIAGYWEDREVKRSIDKWMSAAVAYIESRHIKVARFGDNMRNVAVTEGDKIEAQIQLGWSVDGYGIGDLVTEINAVSEQSLSELISEYEELYEWPEGEAARESVKEQARIELGLKRFLSSGGYTAFTTTFEDLHGMKQLPGLAVQRLMAEGYGFGGEGDWKTAALVRMMKMMAGGKETSFMEDYTYHFEPGNEMILGSHMLEVCPSIAEHKPRIEVHPLSMGAKDDPARLVFDGIAGPAVNVSLIDLGGRFRLVINKVEAVKVPHDMPNLPVARVLWKPQPSLRTSAEAWILAGGAHHTCLSYQLTAEQMLDWAEMSGIEAVLINRDTTILNLRNELKWSEAAYRLRKF

SEQ ID NO: 71 - protein, 509 aa, Bacteroides thetaiotaomicron
  -
MNNVFDQYEVWFVTGAQLLYGGDAVIAVDAHSNEMVNGLNESGKLPVKVVYKGTANSSKEVEAVFKAANNDDKCVGVITWMHTFSPAKMWIHGLQQLKKPLLHLHTQFNKEIPWDTMDMDFMNLNQSAHGDREFGHICTRMRIRRKVVVGYWKEEETLHKIAVWMRVCAGWADSQDMLIIRFGDQMNNVAVTDGDKVEAEQRMGYHVDYCPASELMEYHKDIKNADVDALVATYFNDYDHDASLEDKSTEAYQKVWNAAKAELALRAILKAKGAKGFTTNFDDLGQTDGSYFDQIPGLASQRLMAEGYGFGAEGDWKSAALYRTVWVMNQGLPKGCSFLEDYTLNFDGANSSILQSHMLEICPLIAANKPRLEVHFLGIGIRKSQTARLVFTSKTGTGCTATVVDMGNRFRLIVNDVECIEPKPLPKLPVASALWIPMPNLEVGAGAWILAGGTHHSCFSYDLTAEYWEDYAEIAGIEMVHINKDTTISCFKKELRMNEVYYMLNKALC

SEQ ID NO: 72 - protein, 514 aa, Bacteroides plebeius DSM 17135
  -
TTKTRKMNAFDQYEVWFVTGAQLLYGGDAVIAVDAHSNEMVAGLNASGKLPVKVVYKGTANSSKEVEAVFKAANNEEKCIGVITWMHTFSPAKMWIHGLQQLKKPLLHLHTQFNKEIPWDTMDMDFMNLNQSAHGDREFGHICARMRVRRKVVVGYWKDENTLSKIAVWMRVCAAWADSQDMLILRFGDQMNNVAVTDGDKVEAEQRMGYHVDYCPVSELMSYHKEVKDEEVEALVKTYFNEYDHDAALEDKASEAYQKVWNAAKAELALRAILKAKGAKGFTTNFDDLGQTDGSYFDQIPGLASQRLMAEGYGFGAEGDWKSAALYRTVWVMNQGLPNGCSFLEDYTLNFDGENSSILQAHMLEVCPMIAAKKPRLEVHFLGIGVRKSQTARLVFTSKVGTGCTATVVDMGNRFRLIVNDVECIEPKPLPKLPVASALWKPMPNFEIGAGAWILAGGTHHSCFSYDLTAEYWEDYAEIAGIEMVHINKDTTIDSFKKELRMNEVYYMLNKALC

SEQ ID NO: 73 - protein, 501 aa, Anaerophaga thermohalophila DSM 12881
  -
MHDLKKFEVWFVTGSQHLYGDEALKEVDAHSKKIADALNESSQIPVKVVFKPVVTTPDAIYEVCMQANQKDNCVGLITWMHTFSPAKMWIAGLKALQKPFVHLHTQFNRDIPWSEIDMDFMNLNQSAHGGREFGFIASRMRINRKVVVGHWQDEDVQRQVGVWTRAAVGFHTMKNMKVARFGDNMRNVAVTEGDKVDAQIRFGMDVKGYGICDLVDVIETIGDAEIDALCAEIESNYKVADNLKKGADRHESLRESCRIELGLRKFLDEGGFSAFTTTFEDLHGMKQLPGFAVQRLMADGYGFGAEGDWKTAALTHVMKMMATGLEGGTSFMEDYTYHLDPSGQKVLGAHMLEVCESIAEGTPKVEIHPLGIGGKEDPVRSRFSVAPGPAINASMMDMGNRFRLVVNSVEVVRQPQEMPKLPVSSALWIPKPDLKTGATAWILAGGAHHTVFSKALTAEFMEDFAEMAGMEFLLIDEGTTISEFKKELRWNDLYYHLNRGI

SEQ ID NO: 74 - protein, 496 aa, Thermotoga maritima
  -
MIDLKQYEFWFLVGSQYLYGLETLKKVEQQASKIVDSLNDDPIFPSKIVLKPVLKSSSEITEIFEKANADPKCAGVIVWMHTFSPSKMWIRGLSINKKPLLHLHTQYNREIPWDTIDMDYMNLNQSAHGDREHGFIHARMRLPRKVVVGHWEEKEVREKIAKWMRVACAIQDGRMGQIVRFGDNMREVASTEGDKVEAQIKLGWSINTWGVGELAERVKAVPEREVEELLKEYREKYIMPEDEYSLKAIREQAKIEIALREFLKEKNAVGFTTTFEDLHDLPQLPGLAVQRLMEEGYGFGAEGDWKAAGLVRAIKVMGTSLPGGTSFMEDYTYHLTPGNELVLGAHMLEVCPTIAKEKPRIEVHPLSIGGKADPARLVFDGQEGPAVNASIVDMGNRFRLVVNKVLSVPIERKMPKLPTARVLWKPLPDFKRATTAWILAGGSHHTAFSTAIDVEYLIDWAEALEIEYVVIDENLDLEDFKKELRWNELYWGLLKR

SEQ ID NO: 75 - protein, 501 aa, Chitinophaga pinensis DSM 2588
  -
MIQLKQFEAWFITGSQHLYGEETLKQVAAHAEKIAQSLSNEANIPVRIVFKPVVKTPDEIYRICQEANTAPDCIGVIAWMHTFSPAKMWIGGLKVLQRPLLHLHTQFNRDIPWGDIDMDFMNLNQSAHGDREFGFMMSRMRMDRKVVAGHWQDPDVVAEIGVWLRAAAGWFDWQGARFARIGDNMRQVAVTEGDKVEAELQFGYSVNGYGIGDVVKYINGISDAAIGKLVQEYQDTYTLSAALQKNGAQHASLLEAARIELGLRAFLEEGRFKGFTDTFEDLHGMEQLPGIAVQRLMADGYGFGGEGDWKTAALVRAMKVMGSGLPGGNSFMEDYTYHFDPDNRLVLGAHMLEICSSIASGKASCEIHPLGIGGKADPVRLVFNVASGPAINASVIDMGNRFRLLVNEVEAVAPLHELPKLPVARVLWKPYPDMRTGCAAWIQAGGAHHTCYSQNLGAAHMQDFADMAGIEYVKIGQQTDLYQFRNELRWNDAFYLMKGFK

SEQ ID NO: 76 - protein, 489 aa, Clostridium beijerinckii
  -
MLKVKNYEFWFITGSQHLYGPEVIEQVSDNSKIIVDELNKKDLPYKIVFKTVATDSPSIRKVCNDANNDENCAGIITWMHTFSPAKMWIHGLTELRKPLLHLHTQFNKEIPWGTIDMDFMNLNQAAHGDREFGYIGARLDIARKIVVGHWTDASVSADIAKWMAPAVAFTEGHSIKVARFGDNMRNVAVTDGDRIEAQIKFGWIVDYYGVGDLVKSMDTVTENQIDELMAEYSKLYDIDPKASMDSIREQAKIEIGLRTFLDARGYTAFTTNFEALHGMKQLPGLAVQHLMAEGYGFGAEGDWKTAALLRAMKIMAGGKGTGLMEDYTYNMDSENGLILGAHMLEICPTLAATKPVIEVHPLGIGGKEDPARLVFKGASGPAVAASLIDMGNRFRLIVNSVDCVEVTEDMPNLPVASVLWKPQPSLKEGAKAWIMAGGAHHTSFSFYVDEEQLLDWADMVGVECVVINNDTKLSTFKNELKFSSTAWKF

SEQ ID NO: 77 - protein, 495 aa, Halorhabdus utahensis DSM 12940
  -
MSPIPHGTDFDDLEVWFLTGSQHLYGEETLDLVAEDAREVAAGLDDDDRIPVSVEFKSVLTTADAIESVVREANASEDCIGLITWMHTFSPAKMWIRGLQALDVPFVHLHTQFNRELPYDEIDMDFMNANQSAHGGREFGHIVSRLDIDRKVVVGHWEDDDVREQLDTWARAAAARHELRGAKIARFGDNMRDVAVTEGDKVSAQMAFGASVDGYGLGDLVEFVEDVTESEIDDLLEEYDQQYELAAELQADGDRRDSLREAARIELGIRAFLEDGEFVGFTTTFENLTGLSQLPGLAVQRLMADGYGFGPEGDWKSALLTRAMKVMGQGLNGGTSLMEHYTYDLTEGDEKVLGAHMLEICESIAGEQPRLEIHPLDIGGKADPVRAVFDADTGPAINASLVDMGDRFRLITNDVESVGPDEPLPELPVARAVWKPEPDFETAIEAWIKAGGAHHTGYSQAVTNEHLEDFASMTGIEHLHVGADTDIADVERKLS

SEQ ID NO: 78 - protein, 496 aa, Leadbetterella byssophila DSM 17132
  -
MLNLKNFEVWFVTGSQHLYGEETLRQVDEHSKVIADALNQSPHIAVSVVFKPVVKTPEEILQICREANATPNCIGIIAWMHTFSPAKMWIRGLNTLQLPLLHLHTQFNRDIPYADIDMDFMNLNQSAHGDREFGFIMSKLRMPRKVVVGHWQDASVHERINVWSRVAAGVYKMKTMKVARFGDNMRQVAVTDGDKVAAEDKFGFSVNTYAVGDLVSVINQISDTQIDTLLQEYEDTYALMPSLLKGGERRDSLIEAARIELGLKTFLEDGGFSAYTNTFEDLYGMRQLPGIGSQRMMAAGYGYGGEGDWKTSALVHVMKLMASGMKGGNSFMEDYTYHFEPGNEMVLGSHMLEICPSIAEGTVNCEVHPLGIGGKEDPVRLVFNGAPGNALNASLIDLGNRFRLLVNEVEAVKVDKEFPKLPTARVLWKPQPSMEVGLQSWILGGGAHHTVYSQNLTTEYLEDFAEMLGIELLVIGKGTTIRDIKNEIRFNDIAYK

SEQ ID NO: 79 - protein, 501 aa, Muricauda ruestringensis DSM 13258
  -
MKISKKEIWFVTGSQHLYGPETLKQVASNSKDIVDGLNAAEKLPVSLVFKPIVTTPQEITALCREASNSPSCIGVVTWMHTFSPAKMWIAGLKILSKPLCHLHTQFNAEIPWDNIDMDFMNLNQSAHGDREFGFMMSRMRKNRKVVVGHWKDERVQQKLAVWARVALGADELQHMKVARIGDNMREVAVTEGDKVAAQMRFGVAVNGYDSSDITNIIDGLDQKVVDQLIEEYEASYNLSESLQKNGTQRQSLVDSAKIELGLRTFLDDGGFKAFTDTFENLGALKQLPGLAVQRLMADGYGFGGEGDWKTAALTRTMKVMAKGLDGGTSFMEDYTYHFTPEKDYVLGSHMLEICPSIASAKPSCEVHPLGIGGKEDPVRLVFDSPAGEALNASLIDMGNRFRLIVNEVEAVEPMADLPKLPVARVLWDAKPNLDVAATAWIHAGGAHHTVYTQALTTEYMEDFADIFGIELLVIDSDTKLRAFKDQLHANEAYYHLFQHGM

SEQ ID NO: 80 - protein, 429 aa, Paenibacillus lactis
  -
MKLKPHTFWFVTGSQHLYGPETLEQVAEHSRIVAADFDKDPVFPFPIVFKPIVTTPDEIYQLILEANNDETCAGIMTWMHTFSPAKMWIAGLSQLQKPLLHFHTQFNRDIPWETIDMDFMNLNQSAHGDREYGHIGARLGIARKVVVGHWEDGEVRGAIAGWMRTAAAYAESRRLKVARFGDNMRQVAVTEGDKVEAQIKLGWSVNGYGIGDLVHAMNQVGDDEVKSLLNEYAEQYSITKEGLSDGPVRDSIAYQARIEIGLRRFLEEGGFGAFTTTFEDLHGMEQLPGLAVQRLMEAGYGFGGEGDWKTAALTRVLKVLAGNKSTSFMEDYTYHFEPGNHMILGSHMLEVCPTIALDKPSVEVHPLGIGGKADPARLVFNGQDGPAVNASLVDLGHRFRLLVNVVDGVKVEKPMPKLPIVFADVLVVS

SEQ ID NO: 81 - protein, 501 aa, Serratia odorifera DSM 4582
  -
MDAFKQREVWFVIGSQHLYGPQTLQQVKEHAEQVVNSLNRDAGLPVKLVLKPLVTTPDEITTVCRDANYQQQCLGILTWLHTFSPAKMWIAGLSILNKPLLQFHTQFNAEVPWDSMDMDFMNLNQTAHGGREFGFIGARMRQQHSVITGHWQDRNAHQRIAQWMRVAAARQESQQLKVARFGDNMRQVAVTEGDKVGAQIQFGYAVNAYGIGDLVSVINEVSRGDVDTLIEEYEASYVLSEAVKSNGAKRENLIDAARIELGMKRFLEQGDFHAFTTNFEDLHGMKQLPGLAVQRLMQQGYGFGGEGDWKTAALLRILKVMAGGLDGGTSFMEDYTYHFQPGNDLVVGSHMLEVCPSIAKEQKPLLDIQPLGIGGKADPARLIFSTPAGPAVNASLIDMGDRFRLLVNQVDTVEQPHPLPKLPVARAIWQAQPTLATAAEAWILAGGAHHTVFSQALNADYLRLYAEMHNIEFLLIDNDTTLPAFKNEIRWNEAYYQLNRR

SEQ ID NO: 82 - protein, 504 aa, Opitutus terrae PB90-1
  -
MKLLATPEIWFVCGSQHLYGPGPLKQVAANAQKVAAGLAASKKIPLKIVFKALLTTPDEITNLCIEANSDANCAGLILWMHTFSPAKMWIRGLSTLKKPFCHLHTQFNRDLPWGDIDMDFMNLNQAAHGDREAGFLHTRLRLNRKVVVGHWSDAEVQERIGAWVRAARAWHDWQGAKFARFGDNMRFVAVTEGDKVAAELRFGFSTNGYGVGDLVAKVASEGINDRHVDELCAEYEKRYAVAKELRRGGKRHDSLRYGARIELGLRTFLEEGSFKGFTTTFEDLHGLRQLPGLAVQRLMADGYGFGAEGDWKTAALLRAMKVMGEGLDGGTSFMEDYTYHMNPKGHQVLGAHMLEICSTIAATKPSLEIHPLGIGGKEDPVRLVFDAPAGPALNASLIDMGNRFRLLVNEVTAVKTPKLPKLPVARAVWECQPDFKTACAAWIYAGGAHHTGYSYSVTTEMLEDFANIAGIELAVINADTKLGEFKQTLRNNEVYYHLAQGIRV

SEQ ID NO: 83 - protein, 518 aa, Bifidobacterium gallicum DSM 20093
  -
MRTVGIAKDIIMAMDNPFEGKEIWFGVGSQDLYGEEALRQVAEQSTQIVDALNASGLIPVTLVLKPTLKSSDGVRQFMIDASANERCIGVITWMHTFSPAKMWIRGLELLKKPLLQLNTQHHLEIPWETIDMDFMNLNQAAHGDREYGYIVSRLGIARKIVVGHYTDPQVARKIGVWARACAGWDASTHMKVMRWGDNMRNVAVTEGDKTEAERVFGASINTWSVNELVAAYEAVPETQVDELIADYQAKYDVAPNLLDPSKDYESLRIAAREEAAMVNMMRANGCTAGVDNFEDLGSLPQLPGVGPQRFPSEYGFGFSAEGDWKTAVLVRIGAVMGYGLEGGASLMEDYSYNLTPGNEMIMGAHMLEVSPSLGTIDKPKLEIHPLGIGGKADPVRLVFTVKPKKNAVVVSMADMRERFRLLLNVVDVVEPLGSLEQLPCARALWKPEPSLDVSAECWLMAGGSHHTCMTTSVGREAWEDFARIAGVELAQIDADTTPRAFERELQLQDIVHRLDNRH

SEQ ID NO: 84 - protein, 504 aa, Yersinia kristensenii ATCC 33638
  -
MEYPMDVFKQSEVWFVVGSQNLYGPKTLQQVMDNAHHVVNSLNNEAGLPIKLVLKPLVTTPDEITTLCREANYNTTCIGIMVWLHTFSPAKMWIGGLSILSKPLLQFHTQFNAQIPWETMDMDFMNLNQTAHGGREFGFIGARMRQQHSVITGHWQDKAAHQRISQWMRVAAAKQESQQLKVARFGDNMREVAVTEGDKVAAQIQFGYSVNAYGIGDLVTVVDAVSKGDIDTLVEEYEATYQLTDAVKLNGNKRENLLDAARIELGMKHFLEQGGFKAFTTNFENLYGLNQLPGLAVQRLMQQGYGFGAEGDWKTAALLRIMKVMGTGLQGGTSFMEDYTYHFQPGNDLVVGSHMLEVCPSIAKEEKPLLDVQYLGIGGKADPARLIFSTPASTALNASLIDMGNRFRLLVSVVDTIEQPHPLPKLPVARAIWQAQPSLATAAEAWIIAGGAHHTVFSQAIGVDELLLYAEMHGIEFLLIDNDTSLPVFKNEIRWNEVYYHLNR

SEQ ID NO: 85 - protein, 533 aa, Actinomyces urogenitalis DSM 15434
  -
MCPPRLCDATPSRREPDHTTISHQERDAMATALPNPFDGKEIWFLTGSQDLYGEATLAQVADQSQQVARWLDEAESIPVKIVWKPVLKDRDSIRTAMLEANADESCIGIIAWMHTFSPAKMWILGIDALAKPLLQLHTQYSAAMPWDTIDMDYMNLNQAAHGDREFGYILSRLGQPRKVVVGHATQPATQAKIGTWVRAAAGWDALHHTRLVRFGDNMRNVAVTEGDKTEAELRLGVSVNTWGVNDLVAVVDAVSEAEVDELIAEYQEAYEIVPELLAGGERHESLRYGACIEAGMRRFLQEAGAAAFTTNFEDLGGLRQLPGLAVQRLMAAGYGFGAEGDWKTAILVRAAKVMGYGLPGGASLMEDYCYEMREGKEKILGAHMLEVCPSLTESKPRLEIHPLGIGDREDPVRLVFDADRGPGIVVAMSDMRERFRLTANVVEVVGPDEPLPKLPVARAVWEPAPDFHTSTECWMMSGAAHHTVMSTATTLETWQDLAEIAQMELAVIDESTTTRSFTQNLRLNQVYYRLNQA

SEQ ID NO: 86 - protein, 502 aa, Jonesia denitrificans DSM 20603
  -
MNNPFEGKEIWFLTGSQDLYGEETLAQVAEQSQALVSLIDGADSIPVKVVWKPVLKDSDSIRRAMLDANSDDSCIGLIAWMHTFSPAKMWIRGLDALTVPLLHLHTQANVELPWSTIDMDFMNLNQAAHGDREFAYIQSRMNVQRKIVSGHPSDDTVLSEIAAWSRAAAGWNEAQSMRVARFGDNMRNVAVTEGDKTEAEISLGVSVNTWPVNELVDAVDAVSQSDIDALVAEYEELYDVQEELRRGGDRHDSLRYGAAIEIALRGFLEAGKFGAFTTNFEDLGGLRQLPGLAVQRLMADGYGFGAEGDWKTAVLVRIAKVMGYGLPGGASLMEDYTYDLTPGSELILGAHMLEVCPSLTTDKPRLEIHPLGIGGKEDPVRLVFTADAGPAVVVAMSDMRERFRLVVNVVTNVDAPQELPNLPVARAVWQPEPSFKVSTQAWLLTGAAHHTCMDTAASLDTWLDFAQIAQTELVVIDEKTEIRQFAQELRWNQAYYRLAQGF

SEQ ID NO: 87 - protein, 474 aa, Lactobacillus antri DSM 16041
  -
MLKTPDYEFWFAVGSQPLYGPEALEQVEKDGRKLVDGLNASGKLPYKVVFKLVATTADSITKFMKDANYNDKVAGVMTWMHTFSPAKNWIRGTQLLQKPLLHLATQMLDHIPFDTIDFDYMNLNQSAHGDREYDYINARLGVPEKIVYGWWNDPEVQEEIADWQKVAIAYDMSFKIKIARFGDTMRDVAVTEGDKVAAQIKLGWTVDYWPVAELVAAVNAVSEAEIDEQYKRLEDNYDMVEGDNDHDKYVHSVRYQLREYLGIKHFLDEKGYDAFTTNFQDLEGLEQLPGLAVQLLMIDGYGFGAEGDFKSAGLSRLLKIAAENKETAFMEDYTLDLRAGHQAIMGSHMLEVDPTLASDKPRVEVHPLDIGDKADPARLVFTGSEGEGIDVTLSYFDDGYKFIAYDVDCAKPEKEMPNLPVAKQMWTPKCGLKKGATAWMHNGGGHHTVLSMNLTMDQMATLANLFGIELIDIK

SEQ ID NO: 88 - protein, 474 aa, Leuconostoc mesenteroides subsp. mesenteroides ATCC 8293
  -
MADIKDYKFWFVTGSQFLYGPEVLKQVEEDSKKIIEKLNESGNLPYPIEFKTVGVTAENITEAMKEANYDDSVAGVITWAHTFSPAKNWIRGTQLLNKPLLHLATQMLNNIPYDSIDFDYMNLNQSAHGDREYAFINARLRLNNKIVFGHWADEAVQVQIGKWMDVAVAYEESFKIKVVTFADKMRNVAVTDGDKIEAQIKFGWTVDYWGVGDLVTYVNAIDDADIDNLYIELQDKYDFVAGQNDSEKYEHNVKYQLREYLGIKRFLTDKGYSAFTTNFEDLVGLEQLPGLAAQLLMADGFGFAGEGDWKTAALTRLLKIVSHNQATAFMEDYTLDLRQGHEAILGSHMLEVDPTIASDKPRVEVHPLGIGGKEDPARLVFSGRTGDAVDVTISDFGDEFKLISYDVTGNKPEAETPYLPVAKQLWTPKAGLKAGAEGWLTVGGGHHTTLSFSVDSEQLTDLANLFGVTYVDIK

SEQ ID NO: 89 - protein, 504 aa, Bifidobacterium adolescentis L2-32
  -
MAMENPFEGKEIWFGVGSQDLYGEEALRQVAQQTGEMVDFLNATGKIPAKIVLKPTLKSSDGVKAFMTEASANPNVIGVITWCHTFSPAKMWIRGLEVLTKPLLQLATQHHKEIPWETIDMDFMNLNQAAHGDREFGYIVSRLGIPRKIVVGHYTDPEVAEKVGTWARACAGWDASQNMKVMRWGDNMRNVAVTEGDKTEAERVFGASINTWAVNDLVAAYEKVKDSQVKDLIEDYKAKYDVAPELLDSRYDELFIAAKEEAAMVNMMRENGCTAGVDNFEDLGTLPQLPGVGPQRFPSEYGWGFSAEGDWKTSVLVRIGAVMGYGLEGGASLMEDYSYNFVPGNEFDMGSHMLEVSPSIGTIAKPKLAIYPLGIGGKSDPVRLVFSGKPADAVVVSMADERERFRLLMDEVTIVEPQGSLKNLPCARAVWKPKPDLKTAVQCWITAGGSHHTCMTTSVGREAWEDFARIAGVELAVIDENTNARQFEKELELSEMYHRLNNRH

SEQ ID NO: 90 - protein, 578 aa, Arthrobacter aurescens
  -
MNTSENIPLDEQFVIGVDYGTLSGRAVVVRVSDGAEIGSGVFEYPHAVVTDNLPGSSQRLPADWALQVPNDYRDVLRNAVPAAVADAGINPENVVGIGTDFTACTMVPTTADGTPLNELERFADRPHAFVKLWRHHAAQPQADRINQLAAERGESWLPRYGGLISSEWEFAKGLQLLEEDPEVYGAMEHWVEAADWIVWQLCGSYVRNACTAGYKGIYQDGKYPSQDFLTALNPDFKDFVSEKLEHTIGRLGDAAGYLTEEAAAWTGLPAGIAVAVGNVDAHVSAPAANAVEPGQLVAIMGTSTCHVMNGDVLREVPGMCGVVDGGIVDGLWGYEAGQSGVGDIFGWFTKNGVPPEYHQAAKDKGLGIHEYLTELAEKQAIGEHGLIALDWHSGNRSVLVDHELSGVVVGQTLATKPEDTYRALLEATAFGTRTIVDAFRDSGVPVKEFIVAGGLLKNKFLMQVYADITGLQLSTIGSEQGPALGSAIHAAVAAGKYKDIREAASSMAAAPGAVYTPIPENVAAYEVLFQEYRTLHDYFGRGTNNVMHRLKAIQRAAIQGSSHNGPAAQASTLEGASA

SEQ ID NO: 91 - protein, 567 aa, Clavibacter michiganensis
  -
MPSAPVSTATEAQPGADTESYVVGVDYGTLSGRAVVVRVSDGVELGSGVLDYPHAVMDDTLAATGAQLPPEWALQVPSDYVDVLKQAVPAAIREAGIDPARVIGIGTDFTACTMVPTLADGTPLNEVDGYADRPHAYVKLWKHHAAQSHADRINALAEERGEKWLARYGGLISSEWEFAKGLQLLEEDPELYGLMEHWVEAADWIVWQLTGSYVRNACTAGYKGILQDGEYPTAEFLGALNPDFAEFAEEKVAHEIGQLGSAAGTLSAEAAAWTGLPEGIAVAVGNVDAHVTAPVARAVEPGQMVAIMGTSTCHVMNSDVLTEVPGMCGVVDGGIVSGLYGYEAGQSGVGDIFAWYVKNQVPARYAEEAAAAGKSVHQHLTDLAADQPVGGHGLVALDWHSGNRSVLVDHELSGLVIGTTLTTRTEEVYRALLEATAFGTRKIVETFAASGVPVTEFIVAGGLLKNAFLMQAYSDILRLPISVITSEQGPALGSAIHAAVAAGAYPDVRDAGDAMGKVERGKYQPSEERALAYDRLYAEYSTLHDHFGRGANDVMKRLKSLKREARA

SEQ ID NO: 92 - protein, 565 aa, Gramella forsetii
  -
MSNYVIGLDYGSDSVRAVLVNIDSGKEEASSTHLYKRWKEDKYCEPSINQFRQHPLDHIEGLEKTIKSVLQKTGVEGNSVKAICIDTTGSSPVPVNKDGKALALTEGFEENPNAMMVLWKDHTSINEANEINHLARSWEGEDYTKYEGGIYSSEWFWAKILHIAREDEKVKNAAWSWMEHCDLMTYILIGGSDLESFKRSRCAAGHKAMWHESWGGLPSKDFLSQLDPYLAELKDRLYEKTYTSDEVAGNLSKEWAGKLGLSTECIISVGTFDAHAGAVGAKIDEHSLVRVMGTSTCDIMVARNEEIGKNTVKGICGQVDGSVIPGMIGLEAGQSAFGDVLAWFKDVLSWPLENLVYDSEILAEEQKKKLREEVEDNFIPKLTAQAEKLDLSESMPIALDWVNGRRTPDANQELKSAITNLSLGTKAPHIFNALVNSICFGSKMIVDRFESEGVKINNVIGIGGVARKSAFIMQTLANTLDMPIKVASSDEAPALGAAIYAAVAAGLYPNTIEASKKLGSPFEAEYHPQPEKVKELKKYMAEYRELADFVENKITQKNKQNEFAV

SEQ ID NO: 93 - protein, 533 aa, Lactobacillus plantarum subsp. plantarum ATCC 14917
  -
MNLVETAQAIKTGKVSLGIELGSTRIKAVLITDDFNTIASGSYVWENQFVDGTWTYALEDVWTGIQQSYTQLSADVRSKYHMSLKHINAIGISAMMHGYLAFDQQAKLLVPFRTWRNNITGQAADELTELFDFNIPQRWSIAHLYQAILNNEAHVKQVDFITTLAGYVTWKLSGEKVLGIGDASGVFPIDETTDTYNQTMLTKFSQLDKVKPYSWDIQHILPRVLPAGAIAGKLTAAGASLLDQSGTLDAGSVIAPPEGDAGTGMVGTNSVRKRTGNISVGTSAFSMNVLDKPLSKVYRDIDIVMTPDGSPVAMVHVNNCSSDINAWATIFREFAARLGMELKPDRLYETLFLESTRADADAGGLANYSYQSGENITKIQAGRPLFVRTPNSKFSLPNFMLTQLYAAFAPLQLGMDILVNEEHVQTDVMIAQGGLFRTPVIGQQVLANALNIPITVMSTAGEGGPWGMAVLANFACRQTAMNLEDFLDQEVFKEPESMTLSPEPERVAGYREFIQRYQAGLPVEAAAGQAIKY

SEQ ID NO: 94 - protein, 566 aa, Escherichia coli
  -
MAIAIGLDFGSDSVRALAVDCATGEEIATSVEWYPRWQKGQFCDAPNNQFRHHPRDYIESMEAALKTVLAELSVEQRAAVVGIGVDSTGSTPAPIDADGNVLALRPEFAENPNAMFVLWKDHTAVEEAEEITRLCHAPGNVDYSRYIGGIYSSEWFWAKILHVTRQDSAVAQSAASWIELCDWVPALLSGTTRPQDIRRGRCSAGHKSLWHESWGGLPPASFFDELDPILNRHLPSPLFTDTWTADIPVGTLCPEWAQRLGLPESVVISGGAFDCHMGAVGAGAQPNALVKVIGTSTCDILIADKQSVGERAVKGICGQVDGSVVPGFIGLEAGQSAFGDIYAWFGRVLGWPLEQLAAQHPELKTQINASQKQLLPALTEAWAKNPSLDHLPVVLDWFNGRRTPNANQRLKGVITDLNLATDAPLLFGGLIAATAFGARAIMECFTDQGIAVNNVMALGGIARKNQVIMQACCDVLNRPLQIVASDQCCALGAAIFAAVAAKVHADIPSAQQKMASAVEKTLQPCSEQAQRFEQLYRRYQQWAMSAEQHYLPTSAPAQAAQAVATL

SEQ ID NO: 95 - protein, 553 aa, Opitutus terrae PB90-1
  -
MFTLGLDYGTNSVRALIVRCQDGREFGSAVVNYPSGHQGILLDKHDANLARQHPGDYLFGLEKAVKAALVQARKQRGFSADQIIGIGVDTTGSSPIPVDANNVPLALAKKFAKNLHAQCWLWKDHTSWREAAKITELAAQHRPEYIAKCGNTYSSEWWWSKIWHCLAVDPKVFDAAYSWVELADWVPAVLAGVTDPRQIQRGVCMAGHKALYADEWGGLPDKEFLALLDPKLADLRDRLYEKAHDATVPAGQLSPAWAKKLGLRAGIPIAIGEMDVHYGSIGSGVTEGTLVKVIGTSTCDCGVVSADKQVADIPGICGIVKGAILPGYYGIEAGQSAVGDIFKWWVEVICQGDGALHGKLAAEVAKQPPGHSGLLALDWNNGNRTILVDQRLSGLLLGTTLHTTRAEIYRALIEATAFGARAIIERIRDYGVPIERVVCAGGIARKDPMLMQIYADVTGCTMQVAGSSQACALGSAIGAAVLAGAHRDFTTAQRKMTRIEKKQYRPNPKNQKVYDQLYALYRQIHDAFGGLNKSVDLSRVMKDLLALKDAARA

SEQ ID NO: 96 - protein, 567 aa, Yersinia kristensenii
  -
MTGEVISVDSPIALGLDFGSDSVRVLAVDCQHGIEIDTEVVYYPRWQKGLYSQAAQNQFRHHPLDYIEAMEQAIFQLVSRLSVEQRQHIIGIGVDTTGSTPAPIDKQGQVLALRPDFAENPNAMFVLWKDHTAIEEAEEINRLCSSGEFDDYSRYIGGVYSSEWFWAKILHVTRADQAVCDAAVSWVELCDWIPALLSGTTAPKDIQRGRCGAGHKSLWHPSWGGLPPREFLTALDSRLVDHLDYPMFTETYTAERPVGKITAEWAERLGLPTTVVISGGAFDCHMGAVGAGAQPYTLVKVIGTSTCDILIADKKLVGERAIAGICGQVEGSVVPGWIGMEAGQSAFGDMYAWFSRLLSWPLHQAALAQPELQSQLKLIESTLLASLTAEWAKNPSLDNLPVVLDWFNGRRTPNANQRLKGIITDLNLGTDAPTLFGGFIAATAFGARAIMECFEQQDIPVENILALGGIARKSPVIMQVCADVMNRPLQIVASDQCCALGAAIFAAVAAGIFADVPTAQRHMACKIERTLTPNAAQVARYQQLYQRYQQWCLSAEPHYTPVTKATL

SEQ ID NO: 97 - protein, 540 aa, Bifidobacterium adolescentis L2-32
  -
MTQEQVAVTAEKIRAGKTSLGIEFGSTRIKAVLIDDAYHTIAAGDYEWASHLEDGLWSYTQEEIWKGLQTAYARMAGDVETAYGERLTHVGHIGFSAMMHGYLAFDKSGELLVPFRTWQNTNTHEAHEKLSELFQYNIPERWSVAHLYQAVLNHEEHVSKVDYITTLAGYVHWKLTGEKVLGVGDASGMFPIDPATHTYETEFIKRFDAIEEVAAQPWKLENLLPRPLVAGTPAGTLTAEGAKLLDPTGTLQPGVVLAPPEGDAGTGMVATNSVRVRTGNVSAGTSIFAMVVLEHKLARLHPEVDLVTTPAGDLAGMSHANNFTSDLNAWVGLFGQFAAAIGQPVDAGTLYGTLFRAAIADDVDADCGGLLNYPFRSGEFLAGLPEGRPLFARSPEARMSLGNFMRTQLFSAFSPVKIGMDVMTKDEGVAVDSLVGHGGIFTTPKVAQKILAAAFDTPIKVMATAAEGGAWGMAVLADYLWHADQPLADYLDTRVFADAASTTEAPDANDVAGFEAFFDRFRKGLPIEHAAIESIPLETK

SEQ ID NO: 98 - protein, 504 aa, Clostridium beijerinckii
  -
MEKLLLGIDIGTSACKVAIFDLDGHVVSQANKAYSVYYPEKDFVEQDAEEWWNAVCEATKECIEQSHINPEQIKGIGIDGQGWAALPVDVEGKPLHNAMIWMDRRSTKQCEEVIKKIGEDKIFEVSGNSFDATYTTPKILWLKENKPDVFSKTYKFLQSNSYIAFKLTGAITQDLSQGYGLHCFDMKTGKYDAKLCEELGIPMEKLPDIVPCDQVIGTVNDIAAKQTGLAIGTPVVAGGLDAACGTLGAGVIEFGQTQEQGGQAGGMSICLDKPIGHKKLILGFHVIPNAWLLQGGTVGGGSLKWFRNEFGEYEKHMEEQTGENSFDALVNKAKGVNIGADGVIYLPYMAGERSPIWDKHAKGVFYGLGYDKTKGHIVRAILEGTAYSLEHNLQTAKEVNVDVEELIAIGGAANSLTWTQIKSDVTGKRIKVPTSDTATTLGAAILAGVGTGLYKDYREAVQRTIKITRVHEPNMEAHEIYKRYYPIYLEIYENLKDTFKKSEV

SEQ ID NO: 99 - protein, 529 aa, Actinomyces urogenitalis DSM 15434
  -
MSQHPTTSTPLDLTRTALGIEFGSTRIKAVLIDPAGTVLASGAHDWDNSLVDGVWTYRLEEIITGLRAAYTALANDLKDTHGLALTTTGAIGISGMMHGYIALDAQGQLLTPFRTWRNTITAESSAALSQLFGLNIPQRWTISHLHRAITTAEPHVPHINRVTTLAGYIHWRLTGRHVLGVGEASGVFPIGADGASFDPHMLAAFDQAVSAPWHLAQVLPEVALAGQEAGTLTPDGATLLDPTGTLQPGIPLCPPEGDAGTGMVATAALRPRTGNVSAGTSAFAMIVLDQPLRTLIPEIDLVATPTGRPVAMAHANNCTSDLNAWVEVFSQFATTLGHPIDRGPLFDLLLTAADTTTMDQAGTMSYNFLSGDALVGLTEGRPLTLRRPNAKFGLAGLMRSHLFALFASMAHGVQILRRTTNITIDSMHAHGGIFKTPRIPQQILAAAFNTPVTVSTTASEGGAWGMALLAAYSQWAQNTTLEDWIDNTVSTTQQALTLQATPEQVTEYQHYLEHFINGLPLQKAAIKAF

SEQ ID NO: 100 - protein, 539 aa, Jonesia denitrificans DSM 20603
  -
MTTTPTPHSDIAAAILAGHTSLGIELGSTRIKACLISDDGTPLAEGSHSWENTYDNGLWTYPLPEVDAGMQAAYASLLADTTAQYGVAPTRFGAIGVSAMMHGYLAFDADDNLLVPFRTWRNTNTGPAAGELSELLGYNIPLRWSIAHWYQAILDNEEHVDKVARLTTLAGYVHWKLTGRHVLGVGDASGMFPIDPATRDYDQRLLDLTDTRIATHRSVPAVRNLLPDVLVAGSDAGRLTAQGARWLDTSATLASGIPLCPPEGDAGTGMVATNAVSPRTGNVSAGTSIFAMVVLEQPLTQVHHELDLVTTPTGDLVAMVHCNNGASELNAWATLLGEFAQGLGVTTTPDAIFETFFTAALNGQPDGGGLLAYNYLSGEPITGLEQGRPLFVRTPDSRLTLANFARTHIYGAFGTLALGMRVLSNEGVVIDNMFAHGGMFRTAGVAQRFLAAAINAPVSVGTTAGEGGAWGIAVLAHYTAQRLSGATADDLGTYLTTHIFADSNVTTVEPQPSDVDGFATYLTTYETGLAIERAATTSL

SEQ ID NO: 101 - protein, 534 aa, Lactobacillus antri DSM 16041
  -
MNNSVIKGKIESANTALGIELGSTRIKAVLVTDDYQVVASGDFVWENELRDNIWTYPLEKVWKGIQTSYANLAASVSEQYGIQLTKIGSIGISAMMHGYMPFDQDGNLLVPFRTWRNNITGEAAEKLTKLFNFNIPERWSVAHLYQAILNKEDHVKDIDFITTLDGYVSWRLSGNKNTGIGDASGMFPIDEATKSYDGKMLEQFASLPEVARYPWQIKDILPEVLLAGQPAGKLTEAGAKLLDISGQLQAGSLIAPSEGDAGTGMVATNAVRKRTGNISAGTSAFSMVVLDQKLNKVHRDIDMVTTPDGAPVAMVHTNNCSSDINAWASVFNQFAKALGVNLSPNQLYEKLFDTSLRGDQDAGGLVNFSYLSGENITKVQSGRPMMVRKPDSHFTLANIFKVQLYSAFAPLKIGMDILLREEHIRTDVLIAQGGLFKTPVVAQQVLADALNTPITLMSNAGEGGPWGMAVLALYASDSKGKNLADYLDDEVFVDSESATLYPEPESVQGYEKFIDNYKAALPAEIEAGKDMKLN

SEQ ID NO: 102 - protein, 539 aa, Leuconostoc mesenteroides subsp. mesenteroides ATCC 8293
  -
MADEKIEQAIKNGEVALGVEFGSTTVKAILTTEDFKTIASGSYEWDNSLQDGLWTYAIDDIWLGLQTAYRNLRKKVSVDYNVEIKQINAMGFSAMMHGYLAFDKNNELLVPFRTWRNAITEEASLELTKLFEFNIPQRWSVAHLYQAILNQETHVKNIEFLTTLAGYVHWQLTDQKVIGIGDASGMFPIDEKTGSYSQRMLSQFDSLKSVQQYNWHIQDLLPKPLTAGEVGGYLTEKGARLLDPSGNLSAGATIAPPEGDAGTGMVSTNSVKKRSGNISVGTSIFSMIVLEKSLQHVYTNIDIVTTPTGSPVAMVHANNSASDLSAWVKLFSQFAKMIGSNISTSELYQALFNTALTEAEPDAGGLSGYGYYSGENITAVPEGRPLLVRQPDSEFTIGNLMRFHFFTAFGAIKIGMRILSDEKVLTDNIVAQGGVFKTPIVAQKLLAAALNTDITVMKTAGEGGPWGMAVLSLYTINKKTTQTLDDFLDNNVFINEKYETLSPEPEDVQGFEQFMERYVAGLDIELTAIKTLPSKKEKE

SEQ ID NO: 103 - protein, 531 aa, Bacteroides thetaiotaomicron
  -
MKLDAKSTIETGKAILGIELGSTRIKAVLIDQENKPIAQGSHTWENQLVNGLWTYSIDAIWSGLQDCYADLRSNVKKLYDTEIETLAAIGVSAMMHGYMPFNEKEEILVPFRTWRNTNTGRAAAELSELFVYNIPLRWSISHLYQAILDNEAHVKDIKFLTTLAGYVHWQITGEKVLGIGDASGMLPIDPTTNNYSAEMVAKFNNLIASKEYSWKLEDILPKVLSAGENAGVLTPEGCKKLDASGHLKAGIPVCPPEGDAGTGMVATNAVKQRTGNVSAGTSSFSMIVLEKELSKPYEMIDMVTTPDGSLVAMVHCNNCTSDLNAWVNLFKEYQELLGIPVDMDELYGKLYNIALTGDTDCGGLLSYNYISGEPVTGLAEGRPLFVRSANDKFNLANFMRAHLYASVGVLKIGNDILFNEEKIKVDRITGHGGLFRTKGVGQRVLAAAINSPISVMETAGEGGAWGIALLGSYLVNNKKGQSLADFLDESVFVSDAGVEVSPTPEDVAGFNTYIESYKAGLPIEEAAVKFK

SEQ ID NO: 104 - protein, 472 aa, Escherichia coli
  -
MVTINTESALTPRSLRDTRRMNMFVSVAAAVAGLLFGLDIGVIAGALPFITDHFVLTSRLQEWVVSSMMLGAAIGALFNGWLSFRLGRKYSLMAGAILFVLGSIGSAFATSVEMLIAARVVLGIAVGIASYTAPLYLSEMASENVRGKMISMYQLMVTLGIVLAFLSDTAFSYSGNWRAMLGVLALPAVLLIILVVFLPNSPRWLAEKGRHIEAEEVLRMLRDTSEKAREELNEIRESLKLKQGGWALFKINRNVRRAVFLGMLLQAMQQFTGMNIIMYYAPRIFKMAGFTTTEQQMIATLVVGLTFMFATFIAVFTVDKAGRKPALKIGFSVMALGTLVLGYCLMQFDNGTASSGLSWLSVGMTMMCIAGYAMSAAPVVWILCSEIQPLKCRDFGITCSTTTNWVSNMIIGATFLTLLDSIGAAGTFWLYTALNIAFVGITFWLIPETKNVTLEHIERKLMAGEKLRNIGV

SEQ ID NO: 105 - protein, 522 aa, Candida intermedia
  -
MGLEDNRMVKRFVNVGEKKAGSTAMAIIVGLFAASGGVLFGYDTGTISGVMTMDYVLARYPSNKHSFTADESSLIVSILSVGTFFGALCAPFLNDTLGRRWCLILSALIVFNIGAILQVISTAIPLLCAGRVIAGFGVGLISATIPLYQSETAPKWIRGAIVSCYQWAITIGLFLASCVNKGTEHMTNSGSYRIPLAIQCLWGLILGIGMIFLPETPRFWISKGNQEKAAESLARLRKLPIDHPDSLEELRDITAAYEFETVYGKSSWSQVFSHKNHQLKRLFTGVAIQAFQQLTGVNFIFYYGTTFFKRAGVNGFTISLATNIVNVGSTIPGILLMEVLGRRNMLMGGATGMSLSQLIVAIVGVATSENNKSSQSVLVAFSCIFIAFFAATWGPCAWVVVGELFPLRTRAKSVSLCTASNWLWNWGIAYATPYMVDEDKGNLGSNVFFIWGGFNLACVFFAWYFIYETKGLSLEQVDELYEHVSKAWKSKGFVPSKHSFREQVDQQMDSKTEAIMSEEASV

SEQ ID NO: 106 - protein, 547 aa, Candida intermedia
  -
MSQDSHSSGAATPVNGSILEKEKEDSPVLQVDAPQKGFKDYIVISIFCFMVAFGGFVFGFDTGTISGFVNMSDFKDRFGQHHADGTPYLSDVRVGLMISIFNVGCAVGGIFLCKVADVWGRRIGLMFSMAVYVVGIIIQISSSTKWYQFFIGRLIAGLAVGTVSVVSPLFISEVSPKQIRGTLVCCFQLCITLGIFLGYCTTYGTKTYTDSRQWRIPLGLCFAWAILLVVGMLNMPESPRYLVEKHRIDEAKRSIARSNKIPEEDPFVYTEVQLIQAGIEREALAGQASWKELITGKPKIFRRVIMGIMLQSLQQLTGDNYFFYYGTTIFQAVGLKDSFQTSIILGIVNFASTFVGIYVIERLGRRLCLLTGSAAMFICFIIYSLIGTQHLYKQGYSNETSNTYKASGNAMIFITCLYIFFFASTWAGGVYCIISESYPLRIRSKAMSIATAANWLWGFLISFFTPFITSAIHFYYGFVFTGCLAFSFFYVYFFVYETKGLSLEEVDEMYASGVLPLKSASWVPPNLEHMAHSAGYAGADKATDEQV

SEQ ID NO: 107 - protein, 574 aa, Saccharomyces cerevisiae S288c
  -
MAVEENNMPVVSQQPQAGEDVISSLSKDSHLSAQSQKYSNDELKAGESGSEGSQSVPIEIPKKPMSEYVTVSLLCLCVAFGGFMFGWDTGTISGFVVQTDFLRRFGMKHKDGTHYLSNVRTGLIVAIFNIGCAFGGIILSKGGDMYGRKKGLSIVVSVYIVGIIIQIASINKWYQYFIGRIISGLGVGGIAVLCPMLISEIAPKHLRGTLVSCYQLMITAGIFLGYCTNYGTKSYSNSVQWRVPLGLCFAWSLFMIGALTLVPESPRYLCEVNKVEDAKRSIAKSNKVSPEDPAVQAELDLIMAGIEAEKLAGNASWGELFSTKTKVFQRLLMGVFVQMFQQLTGNNYFFYYGTVIFKSVGLDDSFETSIVIGVVNFASTFFSLWTVENLGHRKCLLLGAATMMACMVIYASVGVTRLYPHGKSQPSSKGAGNCMIVFTCFYIFCYATTWAPVAWVITAESFPLRVKSKCMALASASNWVWGFLIAFFTPFITSAINFYYGYVFMGCLVAMFFYVFFFVPETKGLSLEEIQELWEEGVLPWKSEGWIPSSRRGNNYDLEDLQHDDKPWYKAMLE

SEQ ID NO: 108 - protein, 542 aa, Scheffersomyces stipitis CBS 6054
  -
MSYEDKLVQPALKFRTFLDRLPNIYNVYIIASISCISGMMFGFDISSMSAFIGEDDYKNFFNNPGSDIQGFITSCMALGSFFGSIVSSFISEPFGRRASLLLCSFFWMVGAAVQSSSQNRAQLMIGRIIAGFGVGFGSSVAPVYGSELAPRKIRGFVGGIFQFCVTLGILIMFYICYGLHFINGVGSFRIAWGLQIVPGLVLFVGCFFIPESPRWLAKHGYWDEAEFIVAQIQAKGNREDPDVLIEISEIKDQILIEENLKSFGYVDLFTKKYIRRTLTAIFAQIWQQLTGMNVMMYYIVYIFNMAGYSNNANLVASSIQYVLNTAATVPALFLMDYIGRRRLLIGGAIMMMIFQFGVAGILGKYSVPVPGGLPGNPTVTIQIPEDNKSAARGVIACCYLFVVSFASSWGVGIWVYCSEVWGDSASRQRGAAVSTAANWILNFAIAMYTPSSFKNITWKTYIIYAVFCLVMAIHVYFGFPETKGKRLEEVGQMWDENVPAWRSSSWQPTVPLLSDADLAHKMDVSHKEEQSPDAESSSEEKP

SEQ ID NO: 109 - protein, 551 aa, Kluyveromyces lactis NRRL Y-1140
  -
MSLKNWLLLRDIQYEGTFYKKFPHVYNIYVIGFIACISGLMFGFDIASMSSMIGTDVYKDYFSNPDSLTYGGITASMAGGSFLGSLISPNFSDAFGRKVSLHICAALWIIGAILQCAAQDQAMLIVGRVISGMGIGFGSSAAPVYCSEISPPKIRGTISGLFQFSVTVGIMVLFYIGYGCHFIDGAAAFRITWGLQMVPGLILMVGVFFIPESPRWLANHDRWEETSLIVANIVANGDVNNEQVRFQLEEIKEQVIIDSAAKNFGYKDLFRKKTLPKTIVGVSAQMWQQLCGMNVMMYYIVYIFNMAGYTGNTNLVASSIQYVLNVVMTIPALFLIDKFGRRPVLIIGGIFMFTWLFSVAGILATYSVPAPGGVNGDDTVTIQIPSENTSAANGVIASSYLFVCFFAPTWGIGIWIYCSEIFNNMERAKGSALSAATNWAFNFALAMFVPSAFKNISWKTYIIFGVFSVALTIQTFFMFPETKGKTLEEIDQMWVDNIPAWRTANYIPQLPIVKDEEGNKLGLLGNPQHLEDVHSNEKGLLDRSDSASNSN

SEQ ID NO: 110 - protein, 570 aa, Saccharomyces cerevisiae S288c
  -
MNSTPDLISPQKSNSSNSYELESGRSKAMNTPEGKNESFHDNLSESQVQPAVAPPNTGKGVYVTVSICCVMVAFGGFIFGWDTGTISGFVAQTDFLRRFGMKHHDGSHYLSKVRTGLIVSIFNIGCAIGGIVLAKLGDMYGRRIGLIVVVVIYTIGIIIQIASINKWYQYFIGRIISGLGVGGITVLSPMLISEVAPSEMRGTLVSCYQVMITLGIFLGYCTNFGTKNYSNSVQWRVPLGLCFAWALFMIGGMMFVPESPRYLVEAGRIDEARASLAKVNKCPPDHPYIQYELETIEASVEEMRAAGTASWGELFTGKPAMFQRTMMGIMIQSLQQLTGDNYFFYYGTIVFQAVGLSDSFETSIVFGVVNFFSTCCSLYTVDRFGRRNCLMWGAVGMVCCYVVYASVGVTRLWPNGQDQPSSKGAGNCMIVFACFYIFCFATTWAPIAYVVISECFPLRVKSKCMSIASAANWIWGFLISFFTPFITGAINFYYGYVFMGCMVFAYFYVFFFVPETKGLSLEEVNDMYAEGVLPWKSASWVPVSKRGADYNADDLMHDDQPFYKSLFSRK

SEQ ID NO: 111 - protein, 541 aa, Saccharomyces cerevisiae S288c
  -
MSEFATSRVESGSQQTSIHSTPIVQKLETDESPIQTKSEYTNAELPAKPIAAYWTVICLCLMIAFGGFVFGWDTGTISGFVNQTDFKRRFGQMKSDGTYYLSDVRTGLIVGIFNIGCAFGGLTLGRLGDMYGRRIGLMCVVLVYIVGIVIQIASSDKWYQYFIGRIISGMGVGGIAVLSPTLISETAPKHIRGTCVSFYQLMITLGIFLGYCTNYGTKDYSNSVQWRVPLGLNFAFAIFMIAGMLMVPESPRFLVEKGRYEDAKRSLAKSNKVTIEDPSIVAEMDTIMANVETERLAGNASWGELFSNKGAILPRVIMGIMIQSLQQLTGNNYFFYYGTTIFNAVGMKDSFQTSIVLGIVNFASTFVALYTVDKFGRRKCLLGGSASMAICFVIFSTVGVTSLYPNGKDQPSSKAAGNVMIVFTCLFIFFFAISWAPIAYVIVAESYPLRVKNRAMAIAVGANWIWGFLIGFFTPFITSAIGFSYGYVFMGCLVFSFFYVFFFVCETKGLTLEEVNEMYVEGVKPWKSGSWISKEKRVSEE

SEQ ID NO: 112 - protein, 567 aa, Saccharomyces cerevisiae S288c
  -
MNSTPDLISPQKSSENSNADLPSNSSQVMNMPEEKGVQDDFQAEADQVLTNPNTGKGAYVTVSICCVMVAFGGFVFGWDTGTISGFVAQTDFLRRFGMKHKDGSYYLSKVRTGLIVSIFNIGCAIGGIILAKLGDMYGRKMGLIVVVVIYIIGIIIQIASINKWYQYFIGRIISGLGVGGIAVLSPMLISEVAPKEMRGTLVSCYQLMITLGIFLGYCTNFGTKNYSNSVQWRVPLGLCFAWALFMIGGMTFVPESPRYLVEAGQIDEARASLSKVNKVAPDHPFIQQELEVIEASVEEARAAGSASWGELFTGKPAMFKRTMMGIMIQSLQQLTGDNYFFYYGTTVFNAVGMSDSFETSIVFGVVNFFSTCCSLYTVDRFGRRNCLLYGAIGMVCCYVVYASVGVTRLWPNGEGNGSSKGAGNCMIVFACFYIFCFATTWAPIAYVVISETFPLRVKSKAMSIATAANWLWGFLIGFFTPFITGAINFYYGYVFMGCMVFAYFYVFFFVPETKGLTLEEVNDMYAEGVLPWKSASWVPTSQRGANYDADALMHDDQPFYKKMFGKK

SEQ ID NO: 113 - protein, 576 aa, Saccharomyces cerevisiae S288c
  -
MSEEAAYQEDTAVQNTPADALSPVESDSNSALSTPSNKAERDDMKDFDENHEESNNYVEIPKKPASAYVTVSICCLMVAFGGFVFGWDTGTISGFVAQTDFIRRFGMKHHDGTYYLSKVRTGLIVSIFNIGCAIGGIILAKLGDMYGRKMGLIVVVVIYIIGIIIQIASINKWYQYFIGRIISGLGVGGIAVLSPMLISEVSPKHIRGTLVSCYQLMITLGIFLGYCTNYGTKTYTNSVQWRVPLGLGFAWALFMIGGMTFVPESPRYLVEVGKIEEAKRSIALSNKVSADDPAVMAEVEVVQATVEAEKLAGNASWGEIFSTKTKVFQRLIMGAMIQSLQQLTGDNYFFYYGTTVFTAVGLEDSFETSIVLGIVNFASTFVGIFLVERYGRRRCLLWGAASMTACMVVFASVGVTRLWPNGKKNGSSKGAGNCMIVFTCFYLFCFATTWAPIPFVVNSETFPLRVKSKCMAIAQACNWIWGFLIGFFTPFISGAIDFYYGYVFMGCLVFSYFYVFFFVPETKGLTLEEVNTLWEEGVLPWKSPSWVPPNKRGTDYNADDLMHDDQPFYKKMFGKK

SEQ ID NO: 114 - protein, 592 aa, Saccharomyces cerevisiae S288c
  -
MSELENAHQGPLEGSATVSTNSNSYNEKSGNSTAPGTAGYNDNLAQAKPVSSYISHEGPPKDELEELQKEVDKQLEKKSKSDLLFVSVCCLMVAFGGFVFGWDTGTISGFVRQTDFIRRFGSTRANGTTYLSDVRTGLMVSIFNIGCAIGGIVLSKLGDMYGRKIGLMTVVVIYSIGIIIQIASIDKWYQYFIGRIISGLGVGGITVLAPMLISEVSPKQLRGTLVSCYQLMITFGIFLGYCTNFGTKNYSNSVQWRVPLGLCFAWSIFMIVGMTFVPESPRYLVEVGKIEEAKRSLARANKTTEDSPLVTLEMENYQSSIEAERLAGSASWGELVTGKPQMFRRTLMGMMIQSLQQLTGDNYFFYYGTTIFQAVGLEDSFETAIVLGVVNFVSTFFSLYTVDRFGRRNCLLWGCVGMICCYVVYASVGVTRLWPNGQDQPSSKGAGNCMIVFACFYIFCFATTWAPVAYVLISESYPLRVRGKAMSIASACNWIWGFLISFFTPFITSAINFYYGYVFMGCMVFAYFYVFFFVPETKGLTLEEVNEMYEENVLPWKSTKWIPPSRRTTDYDLDATRNDPRPFYKRMFTKEK

SEQ ID NO: 115 - protein, 570 aa, Saccharomyces cerevisiae S288c
  -
MSQDAAIAEQTPVEHLSAVDSASHSVLSTPSNKAERDEIKAYGEGEEHEPVVEIPKRPASAYVTVSIMCIMIAFGGFVFGWDTGTISGFINQTDFIRRFGMKHKDGTNYLSKVRTGLIVSIFNIGCAIGGIILSKLGDMYGRKVGLIVVVVIYIIGIIIQIASINKWYQYFIGRIISGLGVGGIAVLSPMLISEVSPKHLRGTLVSCYQLMITAGIFLGYCTNFGTKNYSNSVQWRVPLGLCFAWALFMIGGMTFVPESPRYLAEVGKIEEAKRSIAVSNKVAVDDPSVLAEVEAVLAGVEAEKLAGNASWGELFSSKTKVLQRLIMGAMIQSLQQLTGDNYFFYYGTTIFKAVGLSDSFETSIVLGIVNFASTFVGIYVVERYGRRTCLLWGAASMTACMVVYASVGVTRLWPNGQDQPSSKGAGNCMIVFACFYIFCFATTWAPIPYVVVSETFPLRVKSKAMSIATAANWLWGFLIGFFTPFITGAINFYYGYVFMGCLVFMFFYVLLVVPETKGLTLEEVNTMWEEGVLPWKSASWVPPSRRGANYDAEEMAHDDKPLYKRMFSTK

SEQ ID NO: 116 - protein, 570 aa, Saccharomyces cerevisiae S288c
  -
MSQDAAIAEQTPVEHLSAVDSASHSVLSTPSNKAERDEIKAYGEGEEHEPVVEIPKRPASAYVTVSIMCIMIAFGGFVFGWDTGTISGFINQTDFIRRFGMKHKDGTNYLSKVRTGLIVSIFNIGCAIGGIILSKLGDMYGRKVGLIVVVVIYIIGIIIQIASINKWYQYFIGRIISGLGVGGIAVLSPMLISEVSPKHLRGTLVSCYQLMITAGIFLGYCTNFGTKNYSNSVQWRVPLGLCFAWALFMIGGMTFVPESPRYLAEVGKIEEAKRSIAVSNKVAVDDPSVLAEVEAVLAGVEAEKLAGNASWGELFSSKTKVLQRLIMGAMIQSLQQLTGDNYFFYYGTTIFKAVGLSDSFETSIVLGIVNFASTFVGIYVVERYGRRTCLLWGAASMTACMVVYASVGVTRLWPNGQDQPSSKGAGNCMIVFACFYIFCFATTWAPIPYVVVSETFPLRVKSKAMSIATAANWLWGFLIGFFTPFITGAINFYYGYVFMGCLVFMFFYVLLVVPETKGLTLEEVNTMWEEGVLPWKSASWVPPSRRGANYDAEEMTHDDKPLYKRMFSTK

SEQ ID NO: 117 - protein, 479 aa, Corynebacterium glutamicum
  -
MAGHIIRSDSRPIEGVMMTETVQQTKKIPRPYIYFFGSFGGILFGYDIGVMTGALPFLQSDWNIQHEAAIIGWITSSLMLGAVFGGVLAGQLSDKLGRRKMILFSALVFMIFSLGCAVAPDGGWVFLAIVRVFLGLGVGAASALVPAYMSEMAPAKIRGRLSGLNQTMIVSGMLASYIVAYFLRNLHETTAWRLMLGLAAIPALVLFLGVLRLPESPRFLIKNGRIEEARTVLSYIRDNDAIDSELKNIQETAELENAIQAKTRLATLFSGRYRYLVAAGVGVAAFQQFQGANAIFYYIPLIVEKASGTEASNALMWPIIQGVILVLGSLLFMVIADKFNRRTLLTVGGTVMGLSFLFPTFIHMTIPDANPMMIVVFLSIYVAFYSFTWAPLTWVIVGEIFPLAIRGRASGLASSFNWIGSFSVGLLFPIMTAQMTQDAVFAIFGIICILGVLFVRFLVPETRGRTLEEIEAHGTKARV

SEQ ID NO: 118 - protein, 553 aa, Scheffersomyces stipitis
  -
MSSQDIPSGVQTPSNASFLEKDEDKIEEVPQNHDATLVALESKGISEYLLICFFCLLVAFGGFVFGFDTGTISGFVNMSDFLERFGQTRADGTHYLSNVRVGLLVSIFNIGCAIGGIFLSKIGDVYGRRVGIMASMVIYVVGIIVQIASQHAWYQVMIGRAITGLAVGTVSVLSPLFIGESSPKHLRGTLVYCFQLCITLGIFIGYCVTYGTKRLSDSRQWRVPLGLCFLWAIFLVVGMLAMPESPRYLVEKKRIEDAKKSVARSNKLSPEDPSVYTEIQLIQAGIDREAIAGSASWTELITGKPAIFRRVVMGIIMQSLQQLTGVNYFFYYGTTIFQAVGLKDSFQTSIILGVVNFAATFIGIWAIERFGRRSCLLVGSAGMFVCFIIYSTIGSFHLYKDGEYNNDNTYKPSGNALIFITCLFIVFFASTWAGGVYTIISESYPLRIRSKAMAIATAANWVFGFLISFFTPFIVSAIHFKFGYVFSGCLLFSFFYVYFFVVETKGLSLEDVDELYASNVVPWKSSKWVPPSTAAMATEAGYAADEKPVDEHV

SEQ ID NO: 119 - protein, 550 aa, Scheffersomyces stipitis
  -
MSSQDLPSGAQTPIDGSSILEDKVEQSSSSNSQSDLASIPATGIKAYLLVCFFCMLVAFGGFVFGFDTGTISGFLNMSDFLSRFGQDGSEGKYLSDIRVGLIVSIFNIGCAIGGIFLSKIGDVYGRRIGIISAMVVYVVGIIIQISSQDKWYQLTIGRGVTGLAVGTVSVLSPMFISESAPKHLRGTLVYCYQLCITLGIFIGYCVTYGTKDLNDSRQWRVPLGLCFLWAIFLVVGMLAMPESPRFLIEKKRIEEAKKSLARSNKLSPEDPGVYTELQLIQAGIDREAAAGSASWMELITGKPAIFRRVIMGIILQSLQQLTGVNYFFYYGTTIFQAVGLQDSFQTSIILGTVNFLSTFVGIWAIERFGRRQCLLVGSAGMFVCFIIYSVIGTTHLFIDGVVDNDNTRQSSGNAMIFITCLFIFFFACTWAGGVFTIISESYPLRIRSKAMSIATAANWMWGFLISFCTPFIVNAINFKFGFVFTGCLLFSFFYVYFFVSETKGLSLEEVDELYAEGIAPWKSGAWVPPSAQQQMQNSTYGAEAKEQEQV

SEQ ID NO: 120 - protein, 566 aa, Scheffersomyces stipitis
  -
MHGGGDGNDITEIIAARRLQIAGKSGVAGLVANSRSFFIAVFASLGGLVYGYNQGMFGQISGMYSFSKAIGVEKIQDNPTLQGLLTSILELGAWVGVLMNGYIADRLGRKKSVVVGVFFFFIGVIVQAVARGGNYDYILGGRFVVGIGVGILSMVVPLYNAEVSPPEIRGSLVALQQLAITFGIMISYWITYGTNYIGGTGSGQSKASWLVPICIQLVPALLLGVGIFFMPESPRWLMNEDREDECLSVLSNLRSLSKEDTLVQMEFLEMKAQKLFERELSAKYFPHLQDGSAKSNFLIGFNQYKSMITHYPTFKRVAVACLIMTFQQWTGVNFILYYAPFIFSSLGLSGNTISLLASGVVGIVMFLATIPAVLWVDRLGRKPVLISGAIIMGICHFVVAAILGQFGGNFVNHSGAGWVAVVFVWIFAIGFGYSWGPCAWVLVAEVFPLGLRAKGVSIGASSNWLNNFAVAMSTPDFVAKAKFGAYIFLGLMCIFGAAYVQFFCPETKGRTLEEIDELFGDTSGTSKMEKEIHEQKLKEVGLLQLLGEENASESENSKADVYHVEK

SEQ ID NO: 121 - protein, 551 aa, Scheffersomyces stipitis
  -
MREVGILDVAHGNVVTIMMKDPVVFLVILFASLGGLLFGYDQGVISGIVTMESFGAKFPRIFMDADYKGWFVSTFLLCAWFGSIINTPIVDRFGRRDSITISCVIFVIGSAFQCAGINTSMLFGGRAVAGLAVGQLTMVVPMYMSELAPPSVRGGLVVIQQLSITIGIMISYWLDYGTHFIGGTRCAPSHPYQGETFNPNVDVPPGGCYGQSDASWRIPFGVQIAPAVLLGIGMIFFPRSPRWLLSKGRDEEAWSSLKYLRRKSHEDQVEREFAEIKAEVVYEDKYKEKRFPGKTGVALTLTGYWDILTTKSHFKRVFIGSAVMFFQQFIGCNAIIYYAPTIFTQLGMNSTTTSLLGTGLYGIVNCLSTLPAVFLIDRCGRKTLLMAGAIGTFISLVIVGAIVGKYGDRLSEFKTAGRTAIAFIFIYDVNFSYSWAPIGWVLPSEIFPIGIRSNAISITTSSTWMNNFIIGLVTPHMLETMKWGTYIFFAAFAIIAFFFTWLIIPETKGVPLEEMDAVFGDTAALQEKNLVTITSVSESDAKDRNSIEMSE

SEQ ID NO: 122 - protein, 550 aa, Scheffersomyces stipitis
  -
MSSQDLPSGAQTPIDGSSILEDKVEQSSSSNSQSDLASIPATGIKAYLLVCFFCMLVAFGGFVFGFDTGTISGFLNMSDFLSRFGQDGSEGKYLSDIRVGLIVSIFNIGCAIGGIFLSKIGDVYGRRIGIISAMVVYVVGIIIQISSQDKWYQLTIGRGVTGLAVGTVSVLSPMFISESAPKHLRGTLVYCYQLCITLGIFIGYCVTYGTKDLNDSRQWRVPLGLCFLWAIFLVVGMLAMPESPRFLIEKKRIEEAKKSLARSNKLSPEDPGVYTEVQLIQAGIDREAAAGSASWMELITGKPAIFRRVIMGIILQSLQQLTGVNYFFYYGTTIFQAVGLQDSFQTSIILGTVNFLSTFVGIWAIERFGRRQCLLVGSAGMFVCFIIYSVIGTTHLFIDGVVDNDNTRQSSGNAMIFITCLFIFFFACTWAGGVFTIISESYPLRIRSKAMSIATAANWMWGFLISFCTPFIVNAINFKFGFVFTGCLLFSFFYVYFFVSETKGLSLEEVDELYAEGIAPWKSGAWVPPSAQQQMQNSTYGAEAKEQEQV

SEQ ID NO: 123 - protein, 498 aa, Arabidopsis thaliana
  -
MAVGSMNVEEGTKAFPAKLTGQVFLCCVIAAVGGLMFGYDIGISGGVTSMDTFLLDFFPHVYEKKHRVHENNYCKFDDQLLQLFTSSLYLAGIFASFISSYVSRAFGRKPTIMLASIFFLVGAILNLSAQELGMLIGGRILLGFGIGFGNQTVPLFISEIAPARYRGGLNVMFQFLITIGILAASYVNYLTSTLKNGWRYSLGGAAVPALILLIGSFFIHETPASLIERGKDEKGKQVLRKIRGIEDIELEFNEIKYATEVATKVKSPFKELFTKSENRPPLVCGTLLQFFQQFTGINVVMFYAPVLFQTMGSGDNASLISTVVTNGVNAIATVISLLVVDFAGRRCLLMEGALQMTATQMTIGGILLAHLKLVGPITGHAVPLIVLILICVYVSGFAWSWGPLGWLVPSEIYPLEVRNAGYFCAVAMNMVCTFIIGQFFLSALCRFRSLLFFFFGIMNIIMGLFVVFFLPETKGVPIEEMAEKRWKTHPRWKKYFKD

SEQ ID NO: 124 - protein, 514 aa, Arabidopsis thaliana
  -
MVAEEARKEAMAKSVSGGKITYFVVASCVMAAMGGVIFGYDIGVSGGVMSMGPFLKRFFPKVYKLQEEDRRRRGNSNNHYCLFNSQLLTSFTSSLYVSGLIATLLASSVTRSWGRKPSIFLGGVSFLAGAALGGSAQNVAMLIIARLLLGVGVGFANQSVPLYLSEMAPAKYRGAISNGFQLCIGIGFLSANVINYETQNIKHGWRISLATAAIPASILTLGSLFLPETPNSIIQTTGDVHKTELMLRRVRGTNDVQDELTDLVEASSGSDTDSNAFLKLLQRKYRPELVMALVIPFFQQVTGINVVAFYAPVLYRTVGFGESGSLMSTLVTGIVGTSSTLLSMLVVDRIGRKTLFLIGGLQMLVSQVTIGVIVMVADVHDGVIKEGYGYAVVVLVCVYVAGFGWSWGPLGWLVPSEIFPLEIRSVAQSVTVAVSFVFTFAVAQSAPPMLCKFRAGIFFFYGGWLVVMTVAVQLFLPETKNVPIEKVVGLWEKHWFWRRMTSKRDIQETTILSH

SEQ ID NO: 125 - protein, 528 aa, Scheffersomyces stipitis
  -
MGLEDSALLQKYINFGEKKAGSTTMGICVGLFAAFGGILFGYDTGTISGIMAMDYVTARFPSNHQSFSSSESSLIVSILSVGTFFGSLSASFISDRLGRRLTLMISTLIIFNVGIILQTASTSIPLLCVGRVFAGLGVGLISAVIPLYQAETVPKWIRGAVVSCYQWAITLGLLLAAVVNQGTHNRNDSGSYRIPIAIQFLWALILGGGMCLLPETPRFWVSKGDNDRAKDSLRRLRKLPLDHPDLIEEYEEIKANYEYEAQYGSGSWSQVFANKNHQRKRLAMGVGIQALQQLTGINFIFYYGTNFFKGSGIKNEFLIQMATNIVNFGSTVPGILLVEIIGRRKLLLGGSAVMSISQLIVAIVGVAAGEGSTSANKCLVAFVCIFIAAFAATWGPLCWAVIAECYPLTVRQKSISLCTASNWLWNWGIAYATPYMVNSGPGNANLGSKVFFIWGGCNIIGGLFVWYLVYETKGLTLEQIDEMYEKVPKAWQSTRFIPSEHAFTQPSAAASVSSGKAEGVSEVEEASV

SEQ ID NO: 126 - protein, 235 aa, Arthrobacter aurescens
  -
MSSLLESIAKVRRDVCDLHAELTRYELVVWTAGNVSGRIPGHDLMVIKPSGVSYDQLTPELMVVTDLYGTPVRGMNTGSAGTVDWGNPELSPSSDTAAHAYVYRHMPEVGGVVHTHSTYATAWAARGEEIPCVLTMMGDEFGGPIPVGPFALIGDDSIGQGIVETLKNSNSPAVLMQNHGPFTIGKSAREAVKAAVMCEEVARTVHISRQLGEPLPIDQAKIESLYKRYQNVYGR

SEQ ID NO: 127 - protein, 236 aa, Clavibacter michiganensis
  -
MSTYAPEIEVAVARVRSEVSRLHGELVRYGLVVWTGGNVSGRVPGADLFVIKPSGVSYDDLSPENMILCDLDGNVIPDTPGSRNAPSSDTAAHAYVYRNMPEVGGVVHTHSTYAVAWAARREPIPCVITAMADEFGGEIPVGPFAIIGDDSIGRGIVETLTGHRSRAVLMAGHGPFTIGKDAKDAVKAAVMVEDVARTVHISRQLGEPAPLPAEAVDSLFDRYQNVYGQAPQGALK

SEQ ID NO: 128 - protein, 234 aa, Gramella forsetii
  -
MSSQYKDLKKECYDANMQLNALGLVIYTFGNVSAVDREKEVFAIKPSGVPYKDLKPEDIVILDFDNNVIEGEMRPSSDTKTHAYLYKNWKNIGGIAHTHATYSVAWAQSQKDIPIFGTTHADHLTEDIPCAAPMRDDLIEGNYEHNTGIQILDCFEKKGISYEEVPMVLIGNHGPFTWGKDAAKAVYHSKVLEAVAEMAYLTLQINPEAPRLKDSLIKKHYERKHGKDAYYGQN

SEQ ID NO: 129 - protein, 242 aa, Lactobacillus plantarum subsp. plantarum ATCC 14917
  -
MLEALKQEVYEANMQLPKLGLVTFTWGNVSGIDREKGLFVIKPSGVDYGELKPSDLVVVNLQGEVVEGKLNPSSDTPTHTVLYNAFPNIGGIVHTHSPWAVAYAAAQMDVPAMNTTHADTFYGDVPAADALTKEEIEADYEGNTGKTIVKTFQERGLDYEAVPASLVSQHGPFAWGPTPAKAVYNAKVLEVVAEEDYHTAQLTRASSELPQYLLDKHYLRKHGASAYYGQNNAHSKDHAVRK

SEQ ID NO: 130 - protein, 231 aa, Escherichia coli
  -
MLEDLKRQVLEANLALPKHNLVTLTWGNVSAVDRERGVFVIKPSGVDYSVMTADDMVVVSIETGEVVEGTKKPSSDTPTHRLLYQAFPSIGGIVHTHSRHATIWAQAGQSIPATGTTHADYFYGTIPCTRKMTDAEINGEYEWETGNVIVETFEKQGIDAAQMPGVLVHSHGPFAWGKNAEDAVHNAIVLEEVAYMGIFCRQLAPQLPDMQQTLLDKHYLRKHGAKAYYGQ

SEQ ID NO: 131 - protein, 232 aa, Opitutus terrae PB90-1
  -
MLEDLKREAYEANLALPREGLINLTFGNASAIDRAKGIFAIKPSGVDYAALKPADMVLVDLDGKQVEGSLRPSSDTPTHRRLFLAFPSIGGVVHTHSSHATAFAQAGRAIPIFGTTHADYFFGDIPVTRKMTPAEIGGGAYEWETGNVIVELFTQQKLDPQDFPAVLVNRHAPFTWGHNVAKAVEVAVAVECIADMALMSLQLNPSLATIEPELLNKHFKRKHGPGAYYGQR

SEQ ID NO: 132 - protein, 231 aa, Yersinia kristensenii
  -
MLNELKQQVLAANLALPRHNLVTFTWGNVSAVDRHRGLLVIKPSGVEYDVMTVDDMVVVELDSGKVVEGSKKPSSDTDTHRVLYLNFPQIGGIVHTHSRHATIWAQAGLDLPAWGTTHADYFYGTIPCTRLMTPEEIAGRYEWETGNVIVDTFQQRGIKPEDVPAVLVNSHGPFAWGSSADNAVHNAVVLEELAYMGLFSRQLNPQLADMQPQLLDKHYLRKHGKNAYYGQ

SEQ ID NO: 133 - protein, 230 aa, Bifidobacterium adolescentis L2-32
  -
MATLADYGPEVRAEVKQVREVVATLHEQLIKWNLVVWTAGNVSQRLHTADLMVIKPSGLRYEYLTPSSMVVCDLDGNVVDGAEAPSSDTASHAYIYRHMPDVYGVVHTHSTYATAWAATGQNIPCGLTMMGDEFGGPVPVGPFRLIGSEAIGEGVVETLKKYPKSPAVLMQNHGPFTIGKDAEAAVKAAAMTEEVAHTMWAAKQLGDIIPISQEDIDSLNDRYTNVYGQH

SEQ ID NO: 134 - protein, 229 aa, Clostridium beijerinckii
  -
MLEELKKQVLKANLELPAKKLITYTWGNVSGIDRSTGLVVIKPSGVEYDNMTLEDLVVVDLEGNVVEGSLKPSSDTPTHLELYKEFDEIGGIVHTHSTWATIWAQIGRAIPACGTTHADYFYGSIPCTRKMTKEEISRAYEKETGTVIIEEITGNNPLHCPGVVVNDHGPFAWGKNAEEAVHNAVVMEEVAKMAYFTELLSPDNIMDKMLMNKHFLRKHGKNAYYGQSK

SEQ ID NO: 135 - protein, 244 aa, Actinomyces urogenitalis
MTTVPVLAELDDALQAAVAATRERVAALHAELPRWGLVVWTAGNVSERVTVDRGNGPEPTDLFVIKPSGVSYDELSAENMVVCTLEGTKIADGTPEHLVPSSDTAAHAYVYRHMEGVGGVVHTHSTYATAWAARREPIPCALTMMGDEFGGEIPIGPFALIGDDSIGRGIVETLRDSKSPAVLMANHGPFTIGKDARAAVKAAVMCEEVAKTVHVARQGGEIHLIPQDLVDRLNDRYQNVYGQH

SEQ ID NO: 136 - protein, 242 aa, Actinomyces urogenitalis
  -
MFNHEQESPRNVPSARGLEGYSQEVLDEIAEVRRIVSTLHAELPKWELVVWTAGNVSQRLKSADLLVIKPSGVTYDELTPEKMVVCDLDGNLVDGDKAPSSDTAAHAYVYRNMPGVYGVVHTHSTYATAWAARAEPIPCVLTMMADEFGGDIPVGPFALIGDDSIGQGIVDTLRESRSRAVLMRNHGPFTIGKDAKDAVKAAVMVEEVARTVHISRQLGEPGRIGQDDIDRLFDRYQNVYGQ

SEQ ID NO: 137 - protein, 242 aa, Leuconostoc mesenteroides subsp. mesenteroides ATCC 8293
  -
MLEKLKNEVYKANMALPKLGLVTFTWGNVSGIDREKGLFVIKPSGIEYDQLKPSDMVVVNLDGEVVEGNLNPSSDTPTHAYLYQHFLNIGGITHTHSPWGVSFAAAKMDIPAVSTTHADTFYGDIPCAPALSEEEIKTAYELNTGKVIVSEFEYRGLDPDATPAALVSQHGPFTWGATPEKSVYNAKVLEVSAEISYHALQSTRSEIHVPQYLLDKHYYRKHGDNAYYGQSSTQSKNHITHA

SEQ ID NO: 138 - protein, 227 aa, Bacteroides thetaiotaomicron
MLEELKEKVFHANLELVKHGLVIFTWGNVSAIDRETELVVIKPSGVSYDDMKAEDMVVVDLDGKVVEGRLKPSSDTPTHVVLYKAFPEIGGVVHTHSTYATAWAQAGCDIPNIGTTHADYFHDAIPCTADMTEAEVKGAYELETGNVIVKRFEGLNPVHTPGVLVKNHGPFSWGKDAHDAVHNAVVMEQVAKMASIAYAVNPNLTMNPLLVEKHFSRKHGPNAYYGQ